European Patent Specification EP 3 739 045 B1, published August 14, 2024. Title: Cellobiohydrolase Variants And Polynucleotides Encoding Same. Applicant: Novozymes A/S Borch, Kim McBrayer, Brett Windahl, Michael Skovbo Westh, Peter Badino, Silke Flindt. The sequence listing filed with the application follows.

SEQUENCE LISTING (85 sequences)

SEQ ID NO: 1 - DNA, 1599 bp, Aspergillus fumigatus
atgctggcctccaccttctcctaccgcatgtacaagaccgcgctcatcctggccgcccttctgggctctggccaggctcagcaggtcggtacttcccaggcggaagtgcatccgtccatgacctggcagagctgcacggctggcggcagctgcaccaccaacaacggcaaggtggtcatcgacgcgaactggcgttgggtgcacaaagtcggcgactacaccaactgctacaccggcaacacctgggacacgactatctgccctgacgatgcgacctgcgcatccaactgcgcccttgagggtgccaactacgaatccacctatggtgtgaccgccagcggcaattccctccgcctcaacttcgtcaccaccagccagcagaagaacattggctcgcgtctgtacatgatgaaggacgactcgacctacgagatgtttaagctgctgaaccaggagttcaccttcgatgtcgatgtctccaacctcccctgcggtctcaacggtgctctgtactttgtcgccatggacgccgacggtggcatgtccaagtacccaaccaacaaggccggtgccaagtacggtactggatactgtgactcgcagtgccctcgcgacctcaagttcatcaacggtcaggccaacgttgaagggtggcagccctcctccaacgatgccaatgcgggtaccggcaaccacgggtcctgctgcgcggagatggatatctgggaggccaacagcatctccacggccttcaccccccatccgtgcgacacgcccggccaggtgatgtgcaccggtgatgcctgcggtggcacctacagctccgaccgctacggcggcacctgcgaccccgacggatgtgatttcaactccttccgccagggcaacaagaccttctacggccctggcatgaccgtcgacaccaagagcaagtttaccgtcgtcacccagttcatcaccgacgacggcacctccagcggcaccctcaaggagatcaagcgcttctacgtgcagaacggcaaggtgatccccaactcggagtcgacctggaccggcgtcagcggcaactccatcaccaccgagtactgcaccgcccagaaaagcctgttccaggaccagaacgtcttcgaaaagcacggcggcctcgagggcatgggtgctgccctcgcccagggcatggttctcgtcatgtccctgtgggatgatcactcggccaacatgctctggctcgacagcaactacccgaccactgcctcttccaccactcccggcgtcgcccgtggtacctgcgacatctcctccggcgtccctgcggatgtcgaggcgaaccaccccgacgcctacgtcgtctactccaacatcaaggtcggccccatcggctcgaccttcaacagcggtggctcgaaccccggtggcggaaccaccacgacaactaccacccagcctactaccaccacgaccacggctggaaaccctggcggcaccggagtcgcacagcactatggccagtgtggtggaatcggatggaccggacccacaacctgtgccagcccttatacctgccagaagctgaatgattattactctcagtgcctgtag

SEQ ID NO: 2 - DNA, 1599 bp, Aspergillus fumigatus; identical to SEQ ID NO: 1

SEQ ID NO: 3 - DNA, 1599 bp, Aspergillus fumigatus
  sig_peptide (1)..(26)
  CDS (1)..(1596)
  mat_peptide (79)..(1596)
atgttggcctccacgttctcctatcgcatgtacaaaacagcgctcatcttggcagccctcttgggctcgggacaggcacagcaggtcggaacctcgcaggccgaggtccatccttccatgacgtggcagtcgtgtacagcgggtggttcgtgtaccacaaacaacggtaaagtcgtgatcgatgcaaactggaggtgggtgcacaaggtcggcgactacaccaactgttacacaggcaacacatgggatacaaccatctgtcccgacgatgccacttgtgcatccaactgtgcactcgagggtgccaactatgagtcgacgtacggagtgaccgcctccggaaactcgctcaggctcaacttcgtcacaacttcccagcagaagaacatcggctcgcggttgtatatgatgaaagacgattccacttacgagatgttcaagctcctcaaccaggaattcactttcgatgtcgacgtctccaacctcccttgtggcttgaacggagcgctctacttcgtcgccatggatgcggatggaggcatgtccaagtatcctaccaacaaagcaggagccaagtatggtacaggttactgtgattcccagtgtcccagggatctcaagttcatcaacggtcaggccaacgtcgagggttggcagccttcgtcgaacgatgccaacgcaggtaccggcaaccacggttcctgttgtgccgaaatggacatttgggaagcgaactcgatctcgacggcgttcactcctcacccgtgtgatacacccggacaggtgatgtgtacaggcgacgcctgtggcggaacctactcgtcggatcgatatggcggtacgtgtgaccccgacggctgtgacttcaactccttcaggcagggcaacaaaacattctatggacctggcatgacggtggatacaaagtcgaaattcacagtcgtcactcagttcatcaccgacgatggtacgtcctcgggtaccttgaaggagatcaaaaggttctatgtccagaacggaaaggtcatcccgaactcggagtccacgtggacaggagtgtcgggtaactccatcactacggagtattgtacagcccagaagtcgctcttccaggatcagaacgtcttcgagaaacatggaggcttggaaggaatgggtgccgcattggcccagggtatggtcctcgtcatgtccttgtgggacgaccactcggccaacatgctctggttggattccaactaccccaccactgcctcgtccacgacaccgggtgtcgcacgcggaacttgtgatatctcctcgggagtgcctgcagacgtcgaggcgaaccatcccgacgcctacgtggtctactcgaacattaaggtgggacccatcggttcgacattcaactccggaggctcgaaccctggaggcggaacgaccactactacaacgactcagccgacaacaacaactaccacagcaggcaaccctggaggtacaggtgtggcccagcactacggacagtgtggcggtatcggatggacaggacctactacttgtgcatcgccttatacctgtcagaaattgaacgactactactcgcagtgtttgtaa

SEQ ID NO: 4 - protein, 532 aa, Aspergillus fumigatus
MLASTFSYRMYKTALILAALLGSGQAQQVGTSQAEVHPSMTWQSCTAGGSCTTNNGKVVIDANWRWVHKVGDYTNCYTGNTWDTTICPDDATCASNCALEGANYESTYGVTASGNSLRLNFVTTSQQKNIGSRLYMMKDDSTYEMFKLLNQEFTFDVDVSNLPCGLNGALYFVAMDADGGMSKYPTNKAGAKYGTGYCDSQCPRDLKFINGQANVEGWQPSSNDANAGTGNHGSCCAEMDIWEANSISTAFTPHPCDTPGQVMCTGDACGGTYSSDRYGGTCDPDGCDFNSFRQGNKTFYGPGMTVDTKSKFTVVTQFITDDGTSSGTLKEIKRFYVQNGKVIPNSESTWTGVSGNSITTEYCTAQKSLFQDQNVFEKHGGLEGMGAALAQGMVLVMSLWDDHSANMLWLDSNYPTTASSTTPGVARGTCDISSGVPADVEANHPDAYVVYSNIKVGPIGSTFNSGGSNPGGGTTTTTTTQPTTTTTTAGNPGGTGVAQHYGQCGGIGWTGPTTCASPYTCQKLNDYYSQCL

SEQ ID NO: 5 - DNA, 1676 bp, Trichoderma reesei
  exon (1)..(461)
  sig_peptide (1)..(17)
  CDS (1)..(461)
  mat_peptide (52)..(1673)
  Intron (462)..(529)
  exon (530)..(1226)
  CDS (530)..(1226)
  Intron (1227)..(1289)
  exon (1290)..(1673)
  CDS (1290)..(1673)
atgtatcggaagttggccgtcatctcggccttcttggccacagctcgtgctcagtcggcctgcactctccaatcggagactcacccgcctctgacatggcagaaatgctcgtctggtggcacgtgcactcaacagacaggctccgtggtcatcgacgccaactggcgctggactcacgctacgaacagcagcacgaactgctacgatggcaacacttggagctcgaccctatgtcctgacaacgagacctgcgcgaagaactgctgtctggacggtgccgcctacgcgtccacgtacggagttaccacgagcggtaacagcctctccattggctttgtcacccagtctgcgcagaagaacgttggcgctcgcctttaccttatggcgagcgacacgacctaccaggaattcaccctgcttggcaacgagttctctttcgatgttgatgtttcgcagctgccgtaagtgacttaccatgaacccctgacgctatcttcttgttggctcccagctgactggccaattcaaggtgcggcttgaacggagctctctacttcgtgtccatggacgcggatggtggcgtgagcaagtatcccaccaacaccgctggcgccaagtacggcacggggtactgtgacagccagtgtccccgcgatctgaagttcatcaatggccaggccaacgttgagggctgggagccgtcatccaacaacgcgaacacgggcattggaggacacggaagctgctgctctgagatggatatctgggaggccaactccatctccgaggctcttaccccccacccttgcacgactgtcggccaggagatctgcgagggtgatgggtgcggcggaacttactccgataacagatatggcggcacttgcgatcccgatggctgcgactggaacccataccgcctgggcaacaccagcttctacggccctggctcaagctttaccctcgataccaccaagaaattgaccgttgtcacccagttcgagacgtcgggtgccatcaaccgatactatgtccagaatggcgtcactttccagcagcccaacgccgagcttggtagttactctggcaacgagctcaacgatgattactgcacagctgaggaggcagaattcggcggatcctctttctcagacaagggcggcctgactcagttcaagaaggctacctctggcggcatggttctggtcatgagtctgtgggatgatgtgagtttgatggacaaacatgcgcgttgacaaagagtcaagcagctgactgagatgttacagtactacgccaacatgctgtggctggactccacctacccgacaaacgagacctcctccacacccggtgccgtgcgcggaagctgctccaccagctccggtgtccctgctcaggtcgaatctcagtctcccaacgccaaggtcaccttctccaacatcaagttcggacccattggcagcaccggcaaccctagcggcggcaaccctcccggcggaaacccgcctggcaccaccaccacccgccgcccagccactaccactggaagctctcccggacctacccagtctcactacggccagtgcggcggtattggctacagcggccccacggtctgcgccagcggcacaacttgccaggtcctgaacccttactactctcagtgcctgtaa

SEQ ID NO: 6 - protein, 514 aa, Trichoderma reesei
MYRKLAVISAFLATARAQSACTLQSETHPPLTWQKCSSGGTCTQQTGSVVIDANWRWTHATNSSTNCYDGNTWSSTLCPDNETCAKNCCLDGAAYASTYGVTTSGNSLSIGFVTQSAQKNVGARLYLMASDTTYQEFTLLGNEFSFDVDVSQLPCGLNGALYFVSMDADGGVSKYPTNTAGAKYGTGYCDSQCPRDLKFINGQANVEGWEPSSNNANTGIGGHGSCCSEMDIWEANSISEALTPHPCTTVGQEICEGDGCGGTYSDNRYGGTCDPDGCDWNPYRLGNTSFYGPGSSFTLDTTKKLTVVTQFETSGAINRYYVQNGVTFQQPNAELGSYSGNELNDDYCTAEEAEFGGSSFSDKGGLTQFKKATSGGMVLVMSLWDDYYANMLWLDSTYPTNETSSTPGAVRGSCSTSSGVPAQVESQSPNAKVTFSNIKFGPIGSTGNPSGGNPPGGNPPGTTTTRRPATTTGSSPGPTQSHYGQCGGIGYSGPTVCASGTTCQVLNPYYSQCL

SEQ ID NO: 7 - DNA, 1374 bp, Thermoascus aurantiacus
  sig_peptide (1)..(17)
  CDS (1)..(1371)
  mat_peptide (52)..(1371)
atgtatcagcgcgctcttctcttctctttcttcctctccgccgcccgcgcgcagcaggccggtaccctaaccgcagagaatcacccttccctgacctggcagcaatgctccagcggcggtagttgtaccacgcagaatggaaaagtcgttatcgatgcgaactggcgttgggtccataccacctctggatacaccaactgctacacgggcaatacgtgggacaccagtatctgtcccgacgacgtgacctgcgctcagaattgtgccttggatggagcggattacagtggcacctatggtgttacgaccagtggcaacgccctgagactgaactttgtcacccaaagctcagggaagaacattggctcgcgcctgtacctgctgcaggacgacaccacttatcagatcttcaagctgctgggtcaggagtttaccttcgatgtcgacgtctccaatctcccttgcgggctgaacggcgccctctactttgtggccatggacgccgacggcggattgtccaaataccctggcaacaaggcaggcgctaagtatggcactggttactgcgactctcagtgccctcgggatctcaagttcatcaacggtcaggccaacgttgaaggctggcagccgtctgccaacgacccaaatgccggcgttggtaaccacggttcctgctgcgctgagatggatgtctgggaagccaacagcatctctactgcggtgacgcctcacccatgcgacacccccggccagaccatgtgccagggagacgactgtggtggaacctactcctccactcgatatgctggtacctgcgaccctgatggctgcgacttcaatccttaccgccagggcaaccactcgttctacggccccgggaagatcgtcgacactagctccaaattcaccgtcgtcacccagttcatcaccgacgacgggaccccctccggcaccctgacggagatcaaacgcttctacgtccagaacggcaaggtgatcccccagtcggagtcgacgatcagcggcgtcaccggcaactcaatcaccaccgagtattgcacggcccagaaggccgccttcggcgacaacaccggcttcttcacgcacggcgggcttcagaagatcagtcaggctctggctcagggcatggtcctcgtcatgagcctgtgggacgatcacgccgccaacatgctctggctggacagcacctacccgactgatgcggacccggacacccctggcgtcgcgcgcggtacctgccccacgacctccggcgtcccggccgacgttgagtcgcagaaccccaattcatatgttatctactccaacatcaaggtcggacccatcaactcgaccttcaccgccaactaa

SEQ ID NO: 8 - protein, 457 aa, Thermoascus aurantiacus
MYQRALLFSFFLSAARAQQAGTLTAENHPSLTWQQCSSGGSCTTQNGKVVIDANWRWVHTTSGYTNCYTGNTWDTSICPDDVTCAQNCALDGADYSGTYGVTTSGNALRLNFVTQSSGKNIGSRLYLLQDDTTYQIFKLLGQEFTFDVDVSNLPCGLNGALYFVAMDADGGLSKYPGNKAGAKYGTGYCDSQCPRDLKFINGQANVEGWQPSANDPNAGVGNHGSCCAEMDVWEANSISTAVTPHPCDTPGQTMCQGDDCGGTYSSTRYAGTCDPDGCDFNPYRQGNHSFYGPGKIVDTSSKFTVVTQFITDDGTPSGTLTEIKRFYVQNGKVIPQSESTISGVTGNSITTEYCTAQKAAFGDNTGFFTHGGLQKISQALAQGMVLVMSLWDDHAANMLWLDSTYPTDADPDTPGVARGTCPTTSGVPADVESQNPNSYVIYSNIKVGPINSTFTAN

SEQ ID NO: 9 - DNA, 1428 bp, Rasamsonia emersonii
  exon (1)..(603)
  sig_peptide (1)..(18)
  CDS (1)..(603)
  mat_peptide (55)..(1425)
  Intron (604)..(663)
  exon (664)..(1425)
  CDS (664)..(1425)
atgcttcgacgggctcttcttctatcctcttccgccatccttgctgtcaaggcacagcaggccggcacggcgacggcagagaaccacccgcccctgacatggcaggaatgcaccgcccctgggagctgcaccacccagaacggggcggtcgttcttgatgcgaactggcgttgggtgcacgatgtgaacggatacaccaactgctacacgggcaatacctggaaccccacgtactgccctgacgacgaaacctgcgcccagaactgtgcgctggacggcgcggattacgagggcacctacggcgtgacttcgtcgggcagctccttgaagctcaatttcgtcaccgggtcgaacgtcggatcccgtctctacctgctgcaggacgactcgacctatcagatcttcaagcttctgaaccgcgagtttacctttgacgtcgatgtctccaatcttccgtgcggattgaacggcgctctgtactttgtcgccatggacgccgacggcggcgtgtccaagtacccgaacaacaaggctggtgccaagtacggaaccgggtattgcgactcccaatgcccacgggacctcaagttcatcgacggcgaggtatgtccagtggtaaaatcgatcgtctcgtgaacttctgctgacaggttcgatctacaggccaacgtcgagggctggcagccgtcttcgaacaacgccaacaccggaattggcgaccatggctcctgctgtgcggagatggatgtctgggaagccaacagcatctccaatgcggtcactccgcacccgtgcgacacgccaggccagacgatgtgctctggcgatgactgcggtggcacatactctaacgatcgctacgcgggaacctgcgatcctgacggctgtgacttcaacccttaccgcatgggcaacacttctttctacgggcctggcaagatcatcgataccaccaagcctttcactgtcgtgacgcagttcctcactgatgatggtacggatactggaactctcagcgagatcaagcgcttctacgtccagaacggcaacgtcattccgcagcccaactcggacatcagtggcgtgaccggcaactcgatcacgacggagttctgtactgctcagaagcaggcctttggcgacacggacgacttctctcagcacggtggcctggccaagatgggagcggccatgcagcagggtatggtcctggtgatgagtttgtgggacgactacgccgcgcagatgctgtggctggattccgactacccgacggatgcggaccccacgacccctggtattgcccgtggaacgtgtccgacggactcgggcgtcccatcggatgtcgagtcgcagagccccaactcctacgtgacctactcgaacatcaagtttggtccgatcaactcgaccttcaccgcttcgtga

SEQ ID NO: 10 - protein, 455 aa, Rasamsonia emersonii
MLRRALLLSSSAILAVKAQQAGTATAENHPPLTWQECTAPGSCTTQNGAVVLDANWRWVHDVNGYTNCYTGNTWNPTYCPDDETCAQNCALDGADYEGTYGVTSSGSSLKLNFVTGSNVGSRLYLLQDDSTYQIFKLLNREFTFDVDVSNLPCGLNGALYFVAMDADGGVSKYPNNKAGAKYGTGYCDSQCPRDLKFIDGEANVEGWQPSSNNANTGIGDHGSCCAEMDVWEANSISNAVTPHPCDTPGQTMCSGDDCGGTYSNDRYAGTCDPDGCDFNPYRMGNTSFYGPGKIIDTTKPFTVVTQFLTDDGTDTGTLSEIKRFYVQNGNVIPQPNSDISGVTGNSITTEFCTAQKQAFGDTDDFSQHGGLAKMGAAMQQGMVLVMSLWDDYAAQMLWLDSDYPTDADPTTPGIARGTCPTDSGVPSDVESQSPNSYVTYSNIKFGPINSTFTAS

SEQ ID NO: 11 - DNA, 1599 bp, Talaromyces leycettanus
  sig_peptide (1)..(25)
  CDS (1)..(1596)
  mat_peptide (76)..(1596)
atggccagcctcttctctttcaagatgtacaaggccgctctggtcctctcctctctccttgcggccacccaggcccagcaggccggcaccctgaccaccgaaacccatccttctctgacctggcagcaatgctctgccggcggcagctgcaccactcagaacggcaaggtcgtcatcgacgccaactggcgctgggttcacagcaccagcggctcgaacaactgctacactggcaacacttgggatgctactctctgccctgacgacgtgacttgcgctgccaactgcgccctggacggcgctgactactcgggcacctacggtgtcaccaccagcggcaactctctgcgcctgaacttcgtcacccaggcgtcgcagaagaacgtcggctctcgtctctatctgatggagaatgacacaacctaccagatcttcaagttgctgaaccaggagttcacctttgacgttgatgtctccaaccttccctgcggtctcaacggtgctctctacctggttgccatggatgccgacggcggcatggccaagtacccaaccaacaaggctggtgcgaagtacggaaccggttactgcgactcccagtgccctcgcgacctgaagttcatcaacggtgaggccaatgttgagggatggcagccttcttccaatgaccccaactctggcattggcaaccacggctcttgctgtgctgagatggacatctgggaggccaacagcatctccaatgcagtcactcctcacccttgcgacaccccgggacaggtcatgtgcaccggcaacaactgtggtggcacttacagcactactcgctatgctggcacttgcgatcctgatggctgcgacttcaacccctaccgcatgggcaaccactccttctacggccccaaacagatcgtcgacaccagctccaagttcactgttgttactcagttcctcaccgatgatggcacctccaccggcaccctcagcgagatcaggcgcttctacgttcagaacggccaggtcatccccaactccgtgtccacgatcagcggcgtctccggcaactccatcaccaccgagttctgcacggcccagaagcaggctttcggcgacactgatgacttcagcaagcacggcggtctgtctggcatgtccgccgccctctcccagggtatggttctcgtcatgagcttgtgggacgaccacgccgccaacatgctctggcttgacagcacctacccgaccaacgccacctcttccacccccggtgccgcccgtggtacttgcgacatctcctccggtgtccccgccgatgttgagtccaacgaccccaacgcctacgtcgtctactccaacatcaaggtcggcccgatcggctctaccttcagcagctctggctctggctctagctccagctccagcaccaccaccaccaccaccgcttccccaaccacgaccacctccagcgcttccagcaccggcactggcgttgctcagcactggggtcagtgcggtggccagggatggaccggtccgaccacctgcgttagcccctacacctgccaggagctgaacccctactactaccagtgcctgtaa

SEQ ID NO: 12 - protein, 532 aa, Talaromyces leycettanus
MASLFSFKMYKAALVLSSLLAATQAQQAGTLTTETHPSLTWQQCSAGGSCTTQNGKVVIDANWRWVHSTSGSNNCYTGNTWDATLCPDDVTCAANCALDGADYSGTYGVTTSGNSLRLNFVTQASQKNVGSRLYLMENDTTYQIFKLLNQEFTFDVDVSNLPCGLNGALYLVAMDADGGMAKYPTNKAGAKYGTGYCDSQCPRDLKFINGEANVEGWQPSSNDPNSGIGNHGSCCAEMDIWEANSISNAVTPHPCDTPGQVMCTGNNCGGTYSTTRYAGTCDPDGCDFNPYRMGNHSFYGPKQIVDTSSKFTVVTQFLTDDGTSTGTLSEIRRFYVQNGQVIPNSVSTISGVSGNSITTEFCTAQKQAFGDTDDFSKHGGLSGMSAALSQGMVLVMSLWDDHAANMLWLDSTYPTNATSSTPGAARGTCDISSGVPADVESNDPNAYVVYSNIKVGPIGSTFSSSGSGSSSSSSTTTTTTASPTTTTSSASSTGTGVAQHWGQCGGQGWTGPTTCVSPYTCQELNPYYYQCL

SEQ ID NO: 13 - DNA, 1599 bp, Talaromyces leycettanus
  sig_peptide (1)..(25)
  CDS (1)..(1596)
  mat_peptide (76)..(1596)
atggcgtcctctctctcttacaggatctacaagaatgctctcatcttctcttctctcctggccgctgcccagggtcagcagattggtacctaccagacggagacccatccgcctctgacctggcagacatgcaccagcggcggcagttgcacgaccaaccaaggctccatcgtcctcgatgccaactggcgctgggtgcacgaggtcggcagcaccaccaactgctacaccggcaatacctgggacacctccatctgcagcacggatacgacctgcgctcagcaatgtgccgtcgatggtgccgactacgagggcacctatggtatcacgaccagcggcagccaggtccgcatcaacttcgtcaccaacaactcgaacggaaagaacgtcggcgcgcgtgtctacatgatggcggacaacacccactaccaaatttaccagctgctgaaccaggagttcacctttgatgtcgacgtgtccaacctgccttgcggcctcaacggtgccctctactttgtggtcatggacgccgatggtggtgtctccaagtatcccaacaacaaggctggtgcccagtacggtgtcggttactgcgactcccagtgtcccagagacctcaaattcatccagggacaggccaacgtcgagggctggcaaccgtcgtccaacaacgccaataccggcctgggcaaccacggctcctgctgtgctgaactggacgtctgggagtcgaacagcatctcccaggccctcactccccacccctgcgacactcccaccaataccctgtgcaccggtgatagctgcggtggcacatacagcagcaaccgttatgcgggcacttgcgatcctgacggctgcgatttcaacccctaccgcttgggcaacaccaccttctacggtcctggcaagactattgacaccaccaaacccttcacggttgtgacgcagttcatcacggatgacggcacttccagcggcaccctgtccgaaattaggcgtttctatgtccagaacggtgttacgtacgcccagcccaactctgacgtcagcggtatcagcggcaatgccatcaacagtgcttactgcactgcggagaacaccgtcttcaacggtgccggcaccttcgcgcagcacggcggcctggctggcatgagccaggccatgtccaccggtatggtcttggtgatgagcctgtgggatgattactatgccgacatgctctggctcgacagcacctacccaaccaacgacaccgcaagcacgcccggtgcggtccgtggaacctgctctacgtcgtccggtgtccccagccaggtcgaatccgccagcccgaacgcctacgtgacctactcgaacatcaaggttggtcccattggctcgactttcaactctggcggctctggctctggcagcagctccagcactaccacgaccactcacgccagcaccacgacgacgtcctccgcctcgtctacgggaactggcgtggcccaacactggggccagtgtggtggacagggctggaccggcccaacaacctgcgtttccccgtacacttgccaggagctgaacccgtactactaccagtgtctgtag

SEQ ID NO: 14 - protein, 532 aa, Talaromyces leycettanus
MASSLSYRIYKNALIFSSLLAAAQGQQIGTYQTETHPPLTWQTCTSGGSCTTNQGSIVLDANWRWVHEVGSTTNCYTGNTWDTSICSTDTTCAQQCAVDGADYEGTYGITTSGSQVRINFVTNNSNGKNVGARVYMMADNTHYQIYQLLNQEFTFDVDVSNLPCGLNGALYFVVMDADGGVSKYPNNKAGAQYGVGYCDSQCPRDLKFIQGQANVEGWQPSSNNANTGLGNHGSCCAELDVWESNSISQALTPHPCDTPTNTLCTGDSCGGTYSSNRYAGTCDPDGCDFNPYRLGNTTFYGPGKTIDTTKPFTVVTQFITDDGTSSGTLSEIRRFYVQNGVTYAQPNSDVSGISGNAINSAYCTAENTVFNGAGTFAQHGGLAGMSQAMSTGMVLVMSLWDDYYADMLWLDSTYPTNDTASTPGAVRGTCSTSSGVPSQVESASPNAYVTYSNIKVGPIGSTFNSGGSGSGSSSSTTTTTHASTTTTSSASSTGTGVAQHWGQCGGQGWTGPTTCVSPYTCQELNPYYYQCL

SEQ ID NO: 15 - DNA, 1507 bp, Talaromyces byssochlamydoides
  exon (1)..(603)
  sig_peptide (1)..(18)
  CDS (1)..(603)
  mat_peptide (55)..(1504)
  Intron (604)..(667)
  exon (668)..(1235)
  CDS (668)..(1235)
  Intron (1236)..(1310)
  exon (1311)..(1504)
  CDS (1311)..(1504)
atgtttcgacgggctcttttcctgtcctcttccgccttccttgctgtcaaagcccagcagatcggcacggtcagtccggagaaccatccgcccctggcatgggagcagtgcactgcccctgggagttgcacgactgtgaatggtgcggtcgtccttgatgcgaactggcgttgggtccacaatgttgggggatacaccaactgctacactggcaatacctgggacaccacgtactgccctgacgacgtgacctgcgcagagaattgtgcgctggatggcgcagattacgagggcacctacggcgtgaccacctcgggcagctccctgaagctcgatttcgtcaccgggtctaacgtcggatctcgtctctacctgttggagaatgattcgacctatcagatcttcaagcttctgaaccaggaattcacctttgacgtcgacgtttccaatcttccgtgcggattaaacggcgctctgtaccttgttaccatggctgctgacggcggggtgtctcagtacccgaataacaaggccggcgcagcgtatggaaccggttattgcgattcccagtgtccaagggacttgaagtttatcgatggccaggtatgtagagctgtaatcacccatgttgtgaaatcactctcctactgacatggtcgatttataggccaacgttgagggctggcagccgtcttcgaacaacgccaatacaggtattggcaaccatggctcctgctgtgcggagatggatatctgggaagccaacagcatctccaatgcggtgactccgcacccatgcgacacacccggccagacaatgtgcgaggggaacgactgtggtggcacgtattccaccaatcgctatgcaggcacctgcgatcctgacggctgcgacttcaacccctaccgcatgggcaaccattctttctacggccctggggagattgtcgatactacccagcccttcactgtcgtgacacagttccttaccgatgatggcacggatactggcactctcagcgagatcaaacgcttctacgtccaaaacgggaaagtcattcctcagccgaactccgacattgccggcgtgactggcaactcgatcaccagcgagttttgcgatgcccagaagacggctttcggcgacattaacaactttgatacacacggcggtctggccagtatgggagctgcgctgcagcagggtatggttctggtgatgagtctgtgggacggtaggtccttgggagacacccggacgttctatatcaaccagaactgccagaactgacgaattaaaacacttttagattacgcggcaaacatgctgtggttggacagcatttatccaacaaatgcatctgctagcactcctggtgctgctcgtggaacctgttcgacgagctccggtgtcccatcgcaagtcgagtcgcagagccccaacgcctacgtgacgtactccaacattaaagttggaccaatcaactcgaccttcaccacttcgtaa

SEQ ID NO: 16 - protein, 455 aa, Talaromyces byssochlamydoides
MFRRALFLSSSAFLAVKAQQIGTVSPENHPPLAWEQCTAPGSCTTVNGAVVLDANWRWVHNVGGYTNCYTGNTWDTTYCPDDVTCAENCALDGADYEGTYGVTTSGSSLKLDFVTGSNVGSRLYLLENDSTYQIFKLLNQEFTFDVDVSNLPCGLNGALYLVTMAADGGVSQYPNNKAGAAYGTGYCDSQCPRDLKFIDGQANVEGWQPSSNNANTGIGNHGSCCAEMDIWEANSISNAVTPHPCDTPGQTMCEGNDCGGTYSTNRYAGTCDPDGCDFNPYRMGNHSFYGPGEIVDTTQPFTVVTQFLTDDGTDTGTLSEIKRFYVQNGKVIPQPNSDIAGVTGNSITSEFCDAQKTAFGDINNFDTHGGLASMGAALQQGMVLVMSLWDDYAANMLWLDSIYPTNASASTPGAARGTCSTSSGVPSQVESQSPNAYVTYSNIKVGPINSTFTTS

SEQ ID NO: 17 - DNA, 1353 bp, Myceliophthora thermophila
  sig_peptide (1)..(20)
  CDS (1)..(1350)
  mat_peptide (61)..(1350)
atgaagcagtacctccagtacctcgcggcgaccctgcccctggtgggcctggccacggcccagcaggcgggtaacctgcagaccgagactcaccccaggctcacttggtccaagtgcacggccccgggatcctgccaacaggtcaacggcgaggtcgtcatcgactccaactggcgctgggtgcacgacgagaacgcgcagaactgctacgacggcaaccagtggaccaacgcttgcagctctgccaccgactgcgccgagaattgcgcgctcgagggtgccgactaccagggcacctatggcgcctcgaccagcggcaatgccctgacgctcaccttcgtcactaagcacgagtacggcaccaacattggctcgcgcctctacctcatgaacggcgcgaacaagtaccagatgttcaccctcaagggcaacgagctggccttcgacgtcgacctctcggccgtcgagtgcggcctcaacagcgccctctacttcgtggccatggaggaggatggcggtgtgtcgagctacccgaccaacacggccggtgctaagttcggcactgggtactgcgacgcccaatgcgcacgcgacctcaagttcgtcggcggcaagggcaacatcgagggctggaagccgtccaccaacgatgccaatgccggtgtcggtccttatggcgggtgctgcgctgagatcgacgtctgggagtcgaacaagtatgctttcgctttcaccccgcacggttgcgagaaccctaaataccacgtctgcgagaccaccaactgcggtggcacctactccgaggaccgcttcgctggtgactgcgatgccaacggctgcgactacaacccctaccgcatgggcaaccaggacttctacggtcccggcttgacggtcgataccagcaagaagttcaccgtcgtcagccagttcgaggagaacaagctcacccagttcttcgtccaggacggcaagaagattgagatccccggccccaaggtcgagggcatcgatgcggacagcgccgctatcacccctgagctgtgcagtgccctgttcaaggccttcgatgaccgtgaccgcttctcggaggttggcggcttcgatgccatcaacacggccctcagcactcccatggtcctcgtcatgtccatctgggatgatcactacgccaatatgctctggctcgactcgagctacccccctgagaaggctggccagcctggcggtgaccgtggcccgtgtcctcaggactctggcgtcccggccgacgttgaggctcagtaccctaatgccaaggtcatctggtccaacatccgcttcggccccatcggctcgactgtcaacgtctaa

SEQ ID NO: 18 - protein, 450 aa, Myceliophthora thermophila
MKQYLQYLAATLPLVGLATAQQAGNLQTETHPRLTWSKCTAPGSCQQVNGEVVIDSNWRWVHDENAQNCYDGNQWTNACSSATDCAENCALEGADYQGTYGASTSGNALTLTFVTKHEYGTNIGSRLYLMNGANKYQMFTLKGNELAFDVDLSAVECGLNSALYFVAMEEDGGVSSYPTNTAGAKFGTGYCDAQCARDLKFVGGKGNIEGWKPSTNDANAGVGPYGGCCAEIDVWESNKYAFAFTPHGCENPKYHVCETTNCGGTYSEDRFAGDCDANGCDYNPYRMGNQDFYGPGLTVDTSKKFTVVSQFEENKLTQFFVQDGKKIEIPGPKVEGIDADSAAITPELCSALFKAFDDRDRFSEVGGFDAINTALSTPMVLVMSIWDDHYANMLWLDSSYPPEKAGQPGGDRGPCPQDSGVPADVEAQYPNAKVIWSNIRFGPIGSTVNV

SEQ ID NO: 19 - DNA, 1590 bp, Chaetomium thermophilum
  sig_peptide (1)..(18)
  CDS (1)..(1587)
  mat_peptide (55)..(1587)
atgatgtacaagaagttcgccgctctcgccgccctcgtggctggcgccgccgcccagcaggcttgctccctcaccactgagacccaccccagactcacttggaagcgctgcacctctggcggcaactgctcgaccgtgaacggcgccgtcaccatcgatgccaactggcgctggactcacaccgtttccggctcgaccaactgctacaccggcaacgagtgggatacctccatctgctctgatggcaagagctgcgcccagacctgctgcgtcgacggcgctgactactcttcgacctatggtatcaccaccagcggtgactccctgaacctcaagttcgtcaccaagcaccagtacggcaccaatgtcggctctcgtgtctacctgatggagaacgacaccaagtaccagatgttcgagctcctcggcaacgagttcaccttcgatgtcgatgtctctaacctgggctgcggtctcaacggtgccctctacttcgtctccatggacgctgatggtggtatgagcaagtactctggcaacaaggctggcgccaagtacggtaccggctactgcgatgctcagtgcccgcgcgaccttaagttcatcaacggcgaggccaacattgagaactggaccccttcgaccaatgatgccaacgccggtttcggccgctatggcagctgctgctctgagatggatatctgggaggccaacaacatggctactgccttcactcctcacccttgcaccattatcggccagagccgctgcgagggcaacagctgcggtggcacctacagctctgagcgctatgctggtgtttgcgatcctgatggctgcgacttcaacgcctaccgccagggcgacaagaccttctacggcaagggcatgaccgtcgacaccaccaagaagatgaccgtcgtcacccagttccacaagaactcggctggcgtcctcagcgagatcaagcgcttctacgttcaggacggcaagatcattgccaacgccgagtccaagatccccggcaaccccggcaactccatcacccaggagtggtgcgatgcccagaaggtcgccttcggtgacatcgatgacttcaaccgcaagggcggtatggctcagatgagcaaggccctcgagggccctatggtcctggtcatgtccgtctgggatgaccactacgccaacatgctctggctcgactcgacctaccccatcgacaaggccggcacccccggcgccgagcgcggtgcttgcccgaccacctccggtgtccctgccgagattgaggcccaggtccccaacagcaacgtcatcttctccaacatccgcttcggccccatcggctcgaccgtccctggcctcgacggcagcactcccagcaacccgaccgccaccgttgctcctcccacttctaccaccagcgtgagaagcagcactactcagatttccaccccgactagccagcccggcggctgcaccacccagaagtggggccagtgcggtggtatcggctacaccggctgcactaactgcgttgctggcactacctgcactgagctcaacccctggtacagccagtgcctgtaa

SEQ ID NO: 20 - protein, 529 aa, Chaetomium thermophilum
MMYKKFAALAALVAGAAAQQACSLTTETHPRLTWKRCTSGGNCSTVNGAVTIDANWRWTHTVSGSTNCYTGNEWDTSICSDGKSCAQTCCVDGADYSSTYGITTSGDSLNLKFVTKHQYGTNVGSRVYLMENDTKYQMFELLGNEFTFDVDVSNLGCGLNGALYFVSMDADGGMSKYSGNKAGAKYGTGYCDAQCPRDLKFINGEANIENWTPSTNDANAGFGRYGSCCSEMDIWEANNMATAFTPHPCTIIGQSRCEGNSCGGTYSSERYAGVCDPDGCDFNAYRQGDKTFYGKGMTVDTTKKMTVVTQFHKNSAGVLSEIKRFYVQDGKIIANAESKIPGNPGNSITQEWCDAQKVAFGDIDDFNRKGGMAQMSKALEGPMVLVMSVWDDHYANMLWLDSTYPIDKAGTPGAERGACPTTSGVPAEIEAQVPNSNVIFSNIRFGPIGSTVPGLDGSTPSNPTATVAPPTSTTSVRSSTTQISTPTSQPGGCTTQKWGQCGGIGYTGCTNCVAGTTCTELNPWYSQCL

SEQ ID NO: 21 - DNA, 1578 bp, Humicola grisea
  sig_peptide (1)..(18)
  CDS (1)..(1575)
  mat_peptide (55)..(1575)
atgcgtaccgccaagttcgccaccctcgccgcccttgtggcctcggccgccgcccagcaggcgtgcagtctcaccaccgagaggcacccttccctctcttggaagaagtgcaccgccggcggccagtgccagaccgtccaggcttccatcactctcgactccaactggcgctggactcaccaggtgtctggctccaccaactgctacacgggcaacaagtgggatactagcatctgcactgatgccaagtcgtgcgctcagaactgctgcgtcgatggtgccgactacaccagcacctatggcatcaccaccaacggtgattccctgagcctcaagttcgtcaccaagggccagcactcgaccaacgtcggctcgcgtacctacctgatggacggcgaggacaagtatcagaccttcgagctcctcggcaacgagttcaccttcgatgtcgatgtctccaacatcggctgcggtctcaacggcgccctgtacttcgtctccatggacgccgatggtggtctcagccgctatcctggcaacaaggctggtgccaagtacggtaccggctactgcgatgctcagtgcccccgtgacatcaagttcatcaacggcgaggccaacattgagggctggaccggctccaccaacgaccccaacgccggcgcgggccgctatggtacctgctgctctgagatggatatctgggaagccaacaacatggctactgccttcactcctcacccttgcaccatcattggccagagccgctgcgagggcgactcgtgcggtggcacctacagcaacgagcgctacgccggcgtctgcgaccccgatggctgcgacttcaactcgtaccgccagggcaataagaccttctacggcaagggcatgaccgtcgacaccaccaagaagatcactgtcgtcacccagttcctcaaggatgccaacggcgatctcggcgaggtcaagcgcttctacgtccaggatggcaagatcatccccaactccgagtccaccatccccggcgtcgagggcaattccatcacccaggactggtgcgaccgccagaaggttgcctttggcgacattgacgacttcaaccgcaagggcggcatgaagcagatgggcaaggccctcgccggccccatggtcctggtcatgtccatctgggatgaccacgcctccaacatgctctggctcgactcgaccttccctgtcgatgccgctggcaagcccggcgccgagcgcggtgcctgcccgaccacctcgggtgtccctgctgaggttgaggccgaggcccccaacagcaacgtcgtcttctccaacatccgcttcggccccatcggctcgaccgttgctggtctccccggcgcgggcaacggcggcaacaacggcggcaaccccccgccccccaccaccaccacctcctcggctccggccaccaccaccaccgccagcgctggccccaaggctggccactggcagcagtgcggcggcatcggcttcactggcccgacccagtgcgaggagccctacacttgcaccaagctcaacgactggtactctcagtgcctgtaa

SEQ ID NO: 22 - protein, 525 aa, Humicola grisea
MRTAKFATLAALVASAAAQQACSLTTERHPSLSWKKCTAGGQCQTVQASITLDSNWRWTHQVSGSTNCYTGNKWDTSICTDAKSCAQNCCVDGADYTSTYGITTNGDSLSLKFVTKGQHSTNVGSRTYLMDGEDKYQTFELLGNEFTFDVDVSNIGCGLNGALYFVSMDADGGLSRYPGNKAGAKYGTGYCDAQCPRDIKFINGEANIEGWTGSTNDPNAGAGRYGTCCSEMDIWEANNMATAFTPHPCTIIGQSRCEGDSCGGTYSNERYAGVCDPDGCDFNSYRQGNKTFYGKGMTVDTTKKITVVTQFLKDANGDLGEVKRFYVQDGKIIPNSESTIPGVEGNSITQDWCDRQKVAFGDIDDFNRKGGMKQMGKALAGPMVLVMSIWDDHASNMLWLDSTFPVDAAGKPGAERGACPTTSGVPAEVEAEAPNSNVVFSNIRFGPIGSTVAGLPGAGNGGNNGGNPPPPTTTTSSAPATTTTASAGPKAGHWQQCGGIGFTGPTQCEEPYTCTKLNDWYSQCL

SEQ ID NO: 23 - DNA, 1560 bp, Rasamsonia emersonii
  sig_peptide (1)..(18)
  CDS (1)..(1557)
  mat_peptide (55)..(1557)
atgttgcgaagggccttgttgctctcgtcctccgcaatcttggcggtcaaggcacagcaggcaggcaccgcaaccgcagagaaccatcctccgctcacttggcaggaatgtacagcacctggctcctgtacaacccagaacggagcggtcgtgctcgatgcgaactggcgctgggtgcacgatgtcaacggatacacaaactgttatacaggtaacacgtggaaccctacgtattgtcccgacgacgaaacgtgtgcccagaactgtgcgttggatggagcagactacgagggaacgtatggcgtgacctcgtccggctcctccttgaagctcaacttcgtcacgggctcgaacgtcggctcccgcttgtacctcctccaggacgactcgacctaccagatcttcaagctcctcaacagggagttcaccttcgacgtcgatgtctccaacttgccctgtggtctcaacggagccttgtacttcgtcgcgatggatgcagacggaggtgtctcgaagtaccccaacaacaaggcaggtgccaagtatggtactggctactgtgattcgcagtgtcctcgcgatctcaagttcattgacggtgaggcgaacgtggaaggatggcagccctcgtccaacaacgcgaacactggcatcggtgatcacggttcgtgttgtgccgagatggacgtctgggaagccaactccatctcgaacgcggtcacaccgcacccgtgtgatactcctggccagactatgtgttccggagatgattgtggaggcacctattcgaacgaccggtatgcaggcacgtgtgacccggatggctgtgacttcaacccgtaccgcatgggcaacacctccttctatggaccgggtaagatcatcgatacaactaagcccttcaccgtcgtcacgcagttcctcacagatgacggcacggacacaggtactttgtcggagatcaaacgcttctacgtccagaacggaaacgtcatcccccagccgaactccgacatttcgggagtcacaggcaactcgattacgaccgagttctgtacagcccagaaacaggcattcggtgacacggatgatttctcccagcacggaggattggcgaaaatgggagccgcaatgcagcagggaatggtcctcgtgatgtcgctctgggacgactatgcagcccagatgttgtggctcgactcggactaccccacagacgccgatcccacgacacccggtatcgcacgaggcacttgtccgacagattccggagtcccgtcggacgtcgagtcccagtcccccaactcgtacgtcacctattcgaacatcaaattcggtcccatcaactcgacattcacagcctcgggtggaaaccctcctggcggaaaccctcctggcacaactacaacacgacggcctgcgactacaacgggttcgtcccctggaccgacccagtcccactacggacagtgtggaggcatcggttattccggtccgaccgtctgtgcgtccggcacaacctgtcaggtcttgaacccttactattcgcagtgtctctaa

SEQ ID NO: 24 - protein, 519 aa, Rasamsonia emersonii
MLRRALLLSSSAILAVKAQQAGTATAENHPPLTWQECTAPGSCTTQNGAVVLDANWRWVHDVNGYTNCYTGNTWNPTYCPDDETCAQNCALDGADYEGTYGVTSSGSSLKLNFVTGSNVGSRLYLLQDDSTYQIFKLLNREFTFDVDVSNLPCGLNGALYFVAMDADGGVSKYPNNKAGAKYGTGYCDSQCPRDLKFIDGEANVEGWQPSSNNANTGIGDHGSCCAEMDVWEANSISNAVTPHPCDTPGQTMCSGDDCGGTYSNDRYAGTCDPDGCDFNPYRMGNTSFYGPGKIIDTTKPFTVVTQFLTDDGTDTGTLSEIKRFYVQNGNVIPQPNSDISGVTGNSITTEFCTAQKQAFGDTDDFSQHGGLAKMGAAMQQGMVLVMSLWDDYAAQMLWLDSDYPTDADPTTPGIARGTCPTDSGVPSDVESQSPNSYVTYSNIKFGPINSTFTASGGNPPGGNPPGTTTTRRPATTTGSSPGPTQSHYGQCGGIGYSGPTVCASGTTCQVLNPYYSQCL

SEQ ID NO: 25 - DNA, 1599 bp, Aspergillus fumigatus
  sig_peptide (1)..(26)
  CDS (1)..(1596)
  mat_peptide (79)..(1596)
atgttggcctccacgttctcctatcgcatgtacaaaacagcgctcatcttggcagccctcttgggctcgggacaggcacagcaggtcggaacctcgcaggccgaggtccatccttccatgacgtggcagtcgtgtacagcgggtggttcgtgtaccacaaacaacggtaaagtcgtgatcgatgcaaactggaggtgggtgcacaagactggcgactacaccaactgttacacaggcaacacatgggatacaaccatctgtcccgacgatgccacttgtgcatccaactgtgcactcgagggtgccaactatgagtcgacgtacggagtgaccgcctccggaaactcgctcaggctcaacttcgtcacaacttcccagcagaagaacatcggctcgcggttgtatatgatgaaagacgattccacttacgagatgttcaagctcctcaaccaggaattcactttcgatgtcgacgtctccaacctcccttgtggcttgaacggagcgctctacttcgtcgccatggatgcggatggaggcatgtccaagtatcctaccaacaaagcaggagccaagtatggtacaggttactgtgattcccagtgtcccagggatctcaagttcatcaacggtcaggccaacgtcgagggttggcagccttcgtcgaacgatgccaacgcaggtaccggcaaccacggttcctgttgtgccgaaatggacatttgggaagcgaactcgatctcgacggcgttcactcctcacccgtgtgatacacccggacaggtgatgtgtacaggcgacgcctgtggcggaacctactcgtcggatcgatatggcggtacgtgtgaccccgacggctgtgacttcaactccttcaggcagggcaacaaaacattctatggacctggcatgacggtggatacaaagtcgaaattcacagtcgtcactcagttcatcaccgacgatggtacgtcctcgggtaccttgaaggagatcaaaaggttctatgtccagaacggaaaggtcatcccgaactcggagtccacgtggacaggagtgtcgggtaactccatcactacggagtattgtacagcccagaagtcgctcttccaggatcagaacgtcttcgagaaacatggaggcttggaaggaatgggtgccgcattggcccagggtatggtcctcgtcatgtccttgtgggacgaccactcggccaacatgctctggttggattccaactaccccaccactgcctcgtccacgacaccgggtgtcgcacgcggaacttgtgatatctcctcgggagtgcctgcagacgtcgaggcgaaccatcccgacgcctacgtggtctactcgaacattaaggtgggacccatcggttcgacattcaactccggaggctcgaaccctggaggcggaacgaccactactacaacgactcagccgacaacaacaactaccacagcaggcaaccctggaggtacaggtgtggcccagcactacggacagtgtggcggtatcggatggacaggacctactacttgtgcatcgccttatacctgtcagaaattgaacgactactactcgcagtgtttgtaa

SEQ ID NO: 26 - protein, 532 aa, Aspergillus fumigatus
MLASTFSYRMYKTALILAALLGSGQAQQVGTSQAEVHPSMTWQSCTAGGSCTTNNGKVVIDANWRWVHKTGDYTNCYTGNTWDTTICPDDATCASNCALEGANYESTYGVTASGNSLRLNFVTTSQQKNIGSRLYMMKDDSTYEMFKLLNQEFTFDVDVSNLPCGLNGALYFVAMDADGGMSKYPTNKAGAKYGTGYCDSQCPRDLKFINGQANVEGWQPSSNDANAGTGNHGSCCAEMDIWEANSISTAFTPHPCDTPGQVMCTGDACGGTYSSDRYGGTCDPDGCDFNSFRQGNKTFYGPGMTVDTKSKFTVVTQFITDDGTSSGTLKEIKRFYVQNGKVIPNSESTWTGVSGNSITTEYCTAQKSLFQDQNVFEKHGGLEGMGAALAQGMVLVMSLWDDHSANMLWLDSNYPTTASSTTPGVARGTCDISSGVPADVEANHPDAYVVYSNIKVGPIGSTFNSGGSNPGGGTTTTTTTQPTTTTTTAGNPGGTGVAQHYGQCGGIGWTGPTTCASPYTCQKLNDYYSQCL

SEQ ID NO: 27 - DNA, 1599 bp, Aspergillus fumigatus
  sig_peptide (1)..(26)
  CDS (1)..(1596)
  mat_peptide (79)..(1596)
atgttggcctccacgttctcctatcgcatgtacaaaacagcgctcatcttggcagccctcttgggctcgggacaggcacagcaggtcggaacctcgcaggccgaggtccatccttccatgacgtggcagtcgtgtacagcgggtggttcgtgtaccacaaacaacggtaaagtcgtgatcgatgcaaactggaggtgggtgcacaaggtcggcgactacaccaactgttacacaggcaacacatgggatacaaccatctgtcccgacgatgccacttgtgcatccaactgtgcactcgagggtgccaactatgagtcgacgtacggagtgaccgcctccggaaactcgctcaggctcaacttcgtcacaacttcccagcagaagaacatcggctcgcggttgtatatgatgaaagacgattccacttacgagatgttcaagctcctcaaccaggaattcactttcgatgtcgacgtctccaacctcccttgtggcttgaacggagcgctctacttcgtcgccatggatgcggatggaggcatgtccaagtatcctaccaacaaagcaggagccaagtatggtacaggttactgtgattcccagtgtcccagggatctcaagttcatcaacggtcaggccaacgtcgagggttggcagccttcgtcgaacgatgccaacgcaggtaccggcaaccacggttcctgttgtgccgaaatggacatttgggaagcgaactcgatctcgacggcgttcactcctcacccgtgtgatacacccggacaggtgatgtgtacaggcgacgcctgtggcggaacctactcgtcggatcgatatggcggtacgtgtgaccccgacggctgtgacttcaaccctttcaggcagggcaacaaaacattctatggacctggcatgacggtggatacaaagtcgaaattcacagtcgtcactcagttcatcaccgacgatggtacgtcctcgggtaccttgaaggagatcaaaaggttctatgtccagaacggaaaggtcatcccgaactcggagtccacgtggacaggagtgtcgggtaactccatcactacggagtattgtacagcccagaagtcgctcttccaggatcagaacgtcttcgagaaacatggaggcttggaaggaatgggtgccgcattggcccagggtatggtcctcgtcatgtccttgtgggacgaccactcggccaacatgctctggttggattccaactaccccaccactgcctcgtccacgacaccgggtgtcgcacgcggaacttgtgatatctcctcgggagtgcctgcagacgtcgaggcgaaccatcccgacgcctacgtggtctactcgaacattaaggtgggacccatcggttcgacattcaactccggaggctcgaaccctggaggcggaacgaccactactacaacgactcagccgacaacaacaactaccacagcaggcaaccctggaggtacaggtgtggcccagcactacggacagtgtggcggtatcggatggacaggacctactacttgtgcatcgccttatacctgtcagaaattgaacgactactactcgcagtgtttgtaa

SEQ ID NO: 28 - protein, 532 aa, Aspergillus fumigatus
MLASTFSYRMYKTALILAALLGSGQAQQVGTSQAEVHPSMTWQSCTAGGSCTTNNGKVVIDANWRWVHKVGDYTNCYTGNTWDTTICPDDATCASNCALEGANYESTYGVTASGNSLRLNFVTTSQQKNIGSRLYMMKDDSTYEMFKLLNQEFTFDVDVSNLPCGLNGALYFVAMDADGGMSKYPTNKAGAKYGTGYCDSQCPRDLKFINGQANVEGWQPSSNDANAGTGNHGSCCAEMDIWEANSISTAFTPHPCDTPGQVMCTGDACGGTYSSDRYGGTCDPDGCDFNPFRQGNKTFYGPGMTVDTKSKFTVVTQFITDDGTSSGTLKEIKRFYVQNGKVIPNSESTWTGVSGNSITTEYCTAQKSLFQDQNVFEKHGGLEGMGAALAQGMVLVMSLWDDHSANMLWLDSNYPTTASSTTPGVARGTCDISSGVPADVEANHPDAYVVYSNIKVGPIGSTFNSGGSNPGGGTTTTTTTQPTTTTTTAGNPGGTGVAQHYGQCGGIGWTGPTTCASPYTCQKLNDYYSQCL

SEQ ID NO: 29 - DNA, 21 bp, Aspergillus oryzae
cccttgtcgatgcgatgtatc

SEQ ID NO: 30 - DNA, 21 bp, Aspergillus oryzae
atcctcaattccgtcggtcga

SEQ ID NO: 31 - DNA, 25 bp, Aspergillus oryzae
gtgatacacccggacaggtgatgtg

SEQ ID NO: 32 - DNA, 25 bp, Aspergillus oryzae
ccatatcgatccgacgagtaggttc

SEQ ID NO: 33 - DNA, 46 bp, Aspergillus fumigatus
aactggaggtgggtgcacaagacaggcgactacaccaactgttaca

SEQ ID NO: 34 - DNA, 33 bp, Aspergillus fumigatus
cttgtgcacccacctccagtttgcatcgatcac

SEQ ID NO: 35 - DNA, 47 bp, Aspergillus fumigatus
cccgacggctgtgacttcaaccctttcaggcagggcaacaaaacatt

SEQ ID NO: 36 - DNA, 32 bp, Aspergillus fumigatus
gttgaagtcacagccgtcggggtcacacgtac

SEQ ID NO: 37 - DNA, 1599 bp, Aspergillus fumigatus
  sig_peptide (1)..(26)
  CDS (1)..(1596)
  mat_peptide (79)..(1596)
atgttggcctccacgttctcctatcgcatgtacaaaacagcgctcatcttggcagccctcttgggctcgggacaggcacagcaggtcggaacctcgcaggccgaggtccatccttccatgacgtggcagtcgtgtacagcgggtggttcgtgtaccacaaacaacggtaaagtcgtgatcgatgcaaactggaggtgggtgcacaaggtcggcgactacaccaactgttacacaggcaacacatgggatacaaccatctgtcccgacgatgccacttgtgcatccaactgtgcactcgagggtgccaactatgagtcgacgtacggagtgaccgcctccggaaactcgctcaggctcaacttcgtcacaacttcccagcagaagaacatcggctcgcggttgtatatgatgaaagacgattccacttacgagatgttcaagctcctcaaccaggaattcactttcgatgtcgacgtctccaacctcccttgtggcttgaacggagcgctctacttcgtcgccatggatgcggatggaggcatgtccaagtatcctaccaacaaagcaggagccaagtatggtacaggttactgtgattcccagtgtcccagggatctcaagttcatcaacggtcaggccaacgtcgagggttggcagccttcgtcgaacgatgccaacgcaggtaccggcaaccacggttcctgttgtgccgaaatggacatttgggaagcgaactcgatctcgacggcgttcactcctcacccgtgtgatacacccggacaggtgatgtgtacaggcgacgcctgtggcggaacctactcgtcggatcgatatggcggtacgtgtgaccccgacggctgtgacttcaactccttcaggcagggcaacaaaacattctatggacctggcatgacggtggatacaaagtcgaaattcacagtcgtcactcagttcatcaccgacgatggtacgtcctcgggtaccttgaaggagatcaaaaggttctatgtccagaacggaaaggtcatcccgaactcggagtccacgtggacaggagtgtcgggtaactccatcactacggagtattgtacagcccagaagtcgctcttccaggatcagaacgtcttcgagaaacatggaggcttggaaggaatgggtgccgcattggcccagggtatggtcctcgtcatgtccttgtgggacgaccactcggccaacatgctctggttggattccaactaccccaccgatgccgatcctacgacaccgggtgtcgcacgcggaacttgtgatatctcctcgggagtgcctgcagacgtcgaggcgaaccatcccgacgcctacgtggtctactcgaacattaaggtgggacccatcggttcgacattcaactccggaggctcgaaccctggaggcggaacgaccactactacaacgactcagccgacaacaacaactaccacagcaggcaaccctggaggtacaggtgtggcccagcactacggacagtgtggcggtatcggatggacaggacctactacttgtgcatcgccttatacctgtcagaaattgaacgactactactcgcagtgtttgtaa

SEQ ID NO: 38 - protein, 532 aa, Aspergillus fumigatus
MLASTFSYRMYKTALILAALLGSGQAQQVGTSQAEVHPSMTWQSCTAGGSCTTNNGKVVIDANWRWVHKVGDYTNCYTGNTWDTTICPDDATCASNCALEGANYESTYGVTASGNSLRLNFVTTSQQKNIGSRLYMMKDDSTYEMFKLLNQEFTFDVDVSNLPCGLNGALYFVAMDADGGMSKYPTNKAGAKYGTGYCDSQCPRDLKFINGQANVEGWQPSSNDANAGTGNHGSCCAEMDIWEANSISTAFTPHPCDTPGQVMCTGDACGGTYSSDRYGGTCDPDGCDFNSFRQGNKTFYGPGMTVDTKSKFTVVTQFITDDGTSSGTLKEIKRFYVQNGKVIPNSESTWTGVSGNSITTEYCTAQKSLFQDQNVFEKHGGLEGMGAALAQGMVLVMSLWDDHSANMLWLDSNYPTDADPTTPGVARGTCDISSGVPADVEANHPDAYVVYSNIKVGPIGSTFNSGGSNPGGGTTTTTTTQPTTTTTTAGNPGGTGVAQHYGQCGGIGWTGPTTCASPYTCQKLNDYYSQCL

SEQ ID NO: 39 - DNA, 54 bp, Aspergillus fumigatus
gttggattccaactaccccaccgatgccgatcctacgacaccgggtgtcgcacg

SEQ ID NO: 40 - DNA, 34 bp, Aspergillus fumigatus
ggtggggtagttggaatccaaccagagcatgttg

SEQ ID NO: 41 - DNA, 1599 bp, Aspergillus fumigatus
  sig_peptide (1)..(26)
  CDS (1)..(1596)
  mat_peptide (79)..(1596)
atgttggcctccacgttctcctatcgcatgtacaaaacagcgctcatcttggcagccctcttgggctcgggacaggcacagcaggtcggaacctcgcaggccgaggtccatccttccatgacgtggcagtcgtgtacagcgggtggttcgtgtaccacaaacaacggtaaagtcgtgatcgatgcaaactggaggtgggtgcacaagacaggcgactacaccaactgttacacaggcaacacatgggatacaaccatctgtcccgacgatgccacttgtgcatccaactgtgcactcgagggtgccaactatgagtcgacgtacggagtgaccgcctccggaaactcgctcaggctcaacttcgtcacaacttcccagcagaagaacatcggctcgcggttgtatatgatgaaagacgattccacttacgagatgttcaagctcctcaaccaggaattcactttcgatgtcgacgtctccaacctcccttgtggcttgaacggagcgctctacttcgtcgccatggatgcggatggaggcatgtccaagtatcctaccaacaaagcaggagccaagtatggtacaggttactgtgattcccagtgtcccagggatctcaagttcatcaacggtcaggccaacgtcgagggttggcagccttcgtcgaacgatgccaacgcaggtaccggcaaccacggttcctgttgtgccgaaatggacatttgggaagcgaactcgatctcgacggcgttcactcctcacccgtgtgatacacccggacaggtgatgtgtacaggcgacgcctgtggcggaacctactcgtcggatcgatatggcggtacgtgtgaccccgacggctgtgacttcaactccttcaggcagggcaacaaaacattctatggacctggcatgacggtggatacaaagtcgaaattcacagtcgtcactcagttcatcaccgacgatggtacgtcctcgggtaccttgaaggagatcaaaaggttctatgtccagaacggaaaggtcatcccgaactcggagtccacgtggacaggagtgtcgggtaactccatcactacggagtattgtacagcccagaagtcgctcttccaggatcagaacgtcttcgagaaacatggaggcttggaaggaatgggtgccgcattggcccagggtatggtcctcgtcatgtccttgtgggacgaccactcggccaacatgctctggttggattccaactaccccaccactgcctcgtccacgacaccgggtgtcgcacgcggaacttgtgatatctcctcgggagtgcctgcagacgtcgaggcgaaccatcccgacgcctacgtggtctactcgaacattaaggtgggacccatcggttcgacattcaactccggaggctcgaaccctggaggcggaacgaccactactacaacgactcagccgacaacaacaactaccacagcaggcaaccctggaggtacaggtgtggcccagcactggggacagtgtggcggtatcggatggacaggacctactacttgtgcatcgccttatacctgtcagaaattgaacgactactactcgcagtgtttgtaa

SEQ ID NO: 42 - protein, 532 aa, Aspergillus fumigatus
MLASTFSYRMYKTALILAALLGSGQAQQVGTSQAEVHPSMTWQSCTAGGSCTTNNGKVVIDANWRWVHKTGDYTNCYTGNTWDTTICPDDATCASNCALEGANYESTYGVTASGNSLRLNFVTTSQQKNIGSRLYMMKDDSTYEMFKLLNQEFTFDVDVSNLPCGLNGALYFVAMDADGGMSKYPTNKAGAKYGTGYCDSQCPRDLKFINGQANVEGWQPSSNDANAGTGNHGSCCAEMDIWEANSISTAFTPHPCDTPGQVMCTGDACGGTYSSDRYGGTCDPDGCDFNSFRQGNKTFYGPGMTVDTKSKFTVVTQFITDDGTSSGTLKEIKRFYVQNGKVIPNSESTWTGVSGNSITTEYCTAQKSLFQDQNVFEKHGGLEGMGAALAQGMVLVMSLWDDHSANMLWLDSNYPTTASSTTPGVARGTCDISSGVPADVEANHPDAYVVYSNIKVGPIGSTFNSGGSNPGGGTTTTTTTQPTTTTTTAGNPGGTGVAQHWGQCGGIGWTGPTTCASPYTCQKLNDYYSQCL

SEQ ID NO: 43 - DNA, 43 bp, Artificial Sequence
  SYNTHETIC PRIMER
gtacaggtgtggcccagcactggggacagtgtggcggtatcgg

SEQ ID NO: 44 - DNA, 31 bp, Artificial Sequence
  SYNTHETIC PRIMER
gtgctgggccacacctgtacctccagggttg

SEQ ID NO: 45 - DNA, 1599 bp, Aspergillus fumigatus
  sig_peptide (1)..(26)
  CDS (1)..(1596)
  mat_peptide (79)..(1596)
atgttggcctccacgttctcctatcgcatgtacaaaacagcgctcatcttggcagccctcttgggctcgggacaggcacagcaggtcggaacctcgcaggccgaggtccatccttccatgacgtggcagtcgtgtacagcgggtggttcgtgtaccacaaacaacggtaaagtcgtgatcgatgcaaactggaggtgggtgcacaagacaggcgactacaccaactgttacacaggcaacacatgggatacaaccatctgtcccgacgatgccacttgtgcatccaactgtgcactcgagggtgccaactatgagtcgacgtacggagtgaccgcctccggaaactcgctcaggctcaacttcgtcacaacttcccagcagaagaacatcggctcgcggttgtatatgatgaaagacgattccacttacgagatgttcaagctcctcaaccaggaattcactttcgatgtcgacgtctccaacctcccttgtggcttgaacggagcgctctacttcgtcgccatggatgcggatggaggcatgtccaagtatcctaccaacaaagcaggagccaagtatggtacaggttactgtgattcccagtgtcccagggatctcaagttcatcaacggtcaggccaacgtcgagggttggcagccttcgtcgaacgatgccaacgcaggtaccggcaaccacggttcctgttgtgccgaaatggacatttgggaagcgaactcgatctcgacggcgttcactcctcacccgtgtgatacacccggacaggtgatgtgtacaggcgacgcctgtggcggaacctactcgtcggatcgatatggcggtacgtgtgaccccgacggctgtgacttcaaccctttcaggcagggcaacaaaacattctatggacctggcatgacggtggatacaaagtcgaaattcacagtcgtcactcagttcatcaccgacgatggtacgtcctcgggtaccttgaaggagatcaaaaggttctatgtccagaacggaaaggtcatcccgaactcggagtccacgtggacaggagtgtcgggtaactccatcactacggagtattgtacagcccagaagtcgctcttccaggatcagaacgtcttcgagaaacatggaggcttggaaggaatgggtgccgcattggcccagggtatggtcctcgtcatgtccttgtgggacgaccactcggccaacatgctctggttggattccaactaccccaccactgcctcgtccacgacaccgggtgtcgcacgcggaacttgtgatatctcctcgggagtgcctgcagacgtcgaggcgaaccatcccgacgcctacgtggtctactcgaacattaaggtgggacccatcggttcgacattcaactccggaggctcgaaccctggaggcggaacgaccactactacaacgactcagccgacaacaacaactaccacagcaggcaaccctggaggtacaggtgtggcccagcactggggacagtgtggcggtatcggatggacaggacctactacttgtgcatcgccttatacctgtcagaaattgaacgactactactcgcagtgtttgtaa

SEQ ID NO: 46 - protein, 532 aa, Aspergillus fumigatus
MLASTFSYRMYKTALILAALLGSGQAQQVGTSQAEVHPSMTWQSCTAGGSCTTNNGKVVIDANWRWVHKTGDYTNCYTGNTWDTTICPDDATCASNCALEGANYESTYGVTASGNSLRLNFVTTSQQKNIGSRLYMMKDDSTYEMFKLLNQEFTFDVDVSNLPCGLNGALYFVAMDADGGMSKYPTNKAGAKYGTGYCDSQCPRDLKFINGQANVEGWQPSSNDANAGTGNHGSCCAEMDIWEANSISTAFTPHPCDTPGQVMCTGDACGGTYSSDRYGGTCDPDGCDFNPFRQGNKTFYGPGMTVDTKSKFTVVTQFITDDGTSSGTLKEIKRFYVQNGKVIPNSESTWTGVSGNSITTEYCTAQKSLFQDQNVFEKHGGLEGMGAALAQGMVLVMSLWDDHSANMLWLDSNYPTTASSTTPGVARGTCDISSGVPADVEANHPDAYVVYSNIKVGPIGSTFNSGGSNPGGGTTTTTTTQPTTTTTTAGNPGGTGVAQHWGQCGGIGWTGPTTCASPYTCQKLNDYYSQCL

SEQ ID NO: 47 - DNA, 1599 bp, Aspergillus fumigatus
  sig_peptide (1)..(26)
  CDS (1)..(1596)
  mat_peptide (79)..(1596)
atgttggcctccacgttctcctatcgcatgtacaaaacagcgctcatcttggcagccctcttgggctcgggacaggcacagcaggtcggaacctcgcaggccgaggtccatccttccatgacgtggcagtcgtgtacagcgggtggttcgtgtaccacaaacaacggtaaagtcgtgatcgatgcaaactggaggtgggtgcacaagacaggcgactacaccaactgttacacaggcaacacatgggatacaaccatctgtcccgacgatgccacttgtgcatccaactgtgcactcgagggtgccaactatgagtcgacgtacggagtgaccgcctccggaaactcgctcaggctcaacttcgtcacaacttcccagcagaagaacatcggctcgcggttgtatatgatgaaagacgattccacttacgagatgttcaagctcctcaaccaggaattcactttcgatgtcgacgtctccaacctcccttgtggcttgaacggagcgctctacttcgtcgccatggatgcggatggaggcatgtccaagtatcctaccaacaaagcaggagccaagtatggtacaggttactgtgattcccagtgtcccagggatctcaagttcatcaacggtcaggccaacgtcgagggttggcagccttcgtcgaacgatgccaacgcaggtaccggcaaccacggttcctgttgtgccgaaatggacatttgggaagcgaactcgatctcgacggcgttcactcctcacccgtgtgatacacccggacaggtgatgtgtacaggcgacgcctgtggcggaacctactcgtcggatcgatatggcggtacgtgtgaccccgacggctgtgacttcaaccctttcaggcagggcaacaaaacattctatggacctggcatgacggtggatacaaagtcgaaattcacagtcgtcactcagttcatcaccgacgatggtacgtcctcgggtaccttgaaggagatcaaaaggttctatgtccagaacggaaaggtcatcccgaactcggagtccacgtggacaggagtgtcgggtaactccatcactacggagtattgtacagcccagaagtcgctcttccaggatcagaacgtcttcgagaaacatggaggcttggaaggaatgggtgccgcattggcccagggtatggtcctcgtcatgtccttgtgggacgaccactcggccaacatgctctggttggattccaactaccccaccgatgccgatcctacgacaccgggtgtcgcacgcggaacttgtgatatctcctcgggagtgcctgcagacgtcgaggcgaaccatcccgacgcctacgtggtctactcgaacattaaggtgggacccatcggttcgacattcaactccggaggctcgaaccctggaggcggaacgaccactactacaacgactcagccgacaacaacaactaccacagcaggcaaccctggaggtacaggtgtggcccagcactggggacagtgtggcggtatcggatggacaggacctactacttgtgcatcgccttatacctgtcagaaattgaacgactactactcgcagtgtttgtaa

SEQ ID NO: 48 - protein, 532 aa, Aspergillus fumigatus
MLASTFSYRMYKTALILAALLGSGQAQQVGTSQAEVHPSMTWQSCTAGGSCTTNNGKVVIDANWRWVHKTGDYTNCYTGNTWDTTICPDDATCASNCALEGANYESTYGVTASGNSLRLNFVTTSQQKNIGSRLYMMKDDSTYEMFKLLNQEFTFDVDVSNLPCGLNGALYFVAMDADGGMSKYPTNKAGAKYGTGYCDSQCPRDLKFINGQANVEGWQPSSNDANAGTGNHGSCCAEMDIWEANSISTAFTPHPCDTPGQVMCTGDACGGTYSSDRYGGTCDPDGCDFNPFRQGNKTFYGPGMTVDTKSKFTVVTQFITDDGTSSGTLKEIKRFYVQNGKVIPNSESTWTGVSGNSITTEYCTAQKSLFQDQNVFEKHGGLEGMGAALAQGMVLVMSLWDDHSANMLWLDSNYPTDADPTTPGVARGTCDISSGVPADVEANHPDAYVVYSNIKVGPIGSTFNSGGSNPGGGTTTTTTTQPTTTTTTAGNPGGTGVAQHWGQCGGIGWTGPTTCASPYTCQKLNDYYSQCL

SEQ ID NO: 49 - DNA, 54 bp, Artificial Sequence; identical to SEQ ID NO: 39
  SYNTHETIC PRIMER

SEQ ID NO: 50 - DNA, 34 bp, Artificial Sequence; identical to SEQ ID NO: 40
  SYNTHETIC PRIMER

SEQ ID NO: 51 - DNA, 1705 bp, Artificial Sequence
  Synthetic DNA encoding a Rasamsonia byssochlamydoides cellobiohydrolase I with Aspergillus fumigatus linker and Aspergillus fumigatus carbohydrate binding module
  exon (1)..(603)
  sig_peptide (1)..(18)
  CDS (1)..(603)
  mat_peptide (55)..(1702)
  Intron (604)..(667)
  exon (668)..(1235)
  CDS (668)..(1235)
  Intron (1236)..(1310)
  exon (1311)..(1702)
  CDS (1311)..(1702)
atgtttcgacgggctcttttcctgtcctcttccgccttccttgctgtcaaagcccagcagatcggcacggtcagtccggagaaccatccgcccctggcatgggagcagtgcactgcccctgggagttgcacgactgtgaatggtgcggtcgtccttgatgcgaactggcgttgggtccacaatgttgggggatacaccaactgctacactggcaatacctgggacaccacgtactgccctgacgacgtgacctgcgcagagaattgtgcgctggatggcgcagattacgagggcacctacggcgtgaccacctcgggcagctccctgaagctcgatttcgtcaccgggtctaacgtcggatctcgtctctacctgttggagaatgattcgacctatcagatcttcaagcttctgaaccaggaattcacctttgacgtcgacgtttccaatcttccgtgcggattaaacggcgctctgtaccttgttaccatggctgctgacggcggggtgtctcagtacccgaataacaaggccggcgcagcgtatggaaccggttattgcgattcccagtgtccaagggacttgaagtttatcgatggccaggtatgtagagctgtaatcacccatgttgtgaaatcactctcctactgacatggtcgatttataggccaacgttgagggctggcagccgtcttcgaacaacgccaatacaggtattggcaaccatggctcctgctgtgcggagatggatatctgggaagccaacagcatctccaatgcggtgactccgcacccatgcgacacacccggccagacaatgtgcgaggggaacgactgtggtggcacgtattccaccaatcgctatgcaggcacctgcgatcctgacggctgcgacttcaacccctaccgcatgggcaaccattctttctacggccctggggagattgtcgatactacccagcccttcactgtcgtgacacagttccttaccgatgatggcacggatactggcactctcagcgagatcaaacgcttctacgtccaaaacgggaaagtcattcctcagccgaactccgacattgccggcgtgactggcaactcgatcaccagcgagttttgcgatgcccagaagacggctttcggcgacattaacaactttgatacacacggcggtctggccagtatgggagctgcgctgcagcagggtatggttctggtgatgagtctgtgggacggtaggtccttgggagacacccggacgttctatatcaaccagaactgccagaactgacgaattaaaacacttttagattacgcggcaaacatgctgtggttggacagcatttatccaacaaatgcatctgctagcactcctggtgctgctcgtggaacctgttcgacgagctccggtgtcccatcgcaagtcgagtcgcagagccccaacgcctacgtgacgtactccaacattaaagttggaccaatcaactcgaccttcaccacttcgggctcgaaccctggaggcggaacgaccactactacaacgactcagccgacaacaacaactaccacagcaggcaaccctggaggtacaggtgtggcccagcactacggacagtgtggcggtatcggatggacaggacctactacttgtgcatcgccttatacctgtcagaaattgaacgactactactcgcagtgtttgtaa

SEQ ID NO: 52 - protein, 521 aa, Artificial Sequence
  Synthetic Construct
MFRRALFLSSSAFLAVKAQQIGTVSPENHPPLAWEQCTAPGSCTTVNGAVVLDANWRWVHNVGGYTNCYTGNTWDTTYCPDDVTCAENCALDGADYEGTYGVTTSGSSLKLDFVTGSNVGSRLYLLENDSTYQIFKLLNQEFTFDVDVSNLPCGLNGALYLVTMAADGGVSQYPNNKAGAAYGTGYCDSQCPRDLKFIDGQANVEGWQPSSNNANTGIGNHGSCCAEMDIWEANSISNAVTPHPCDTPGQTMCEGNDCGGTYSTNRYAGTCDPDGCDFNPYRMGNHSFYGPGEIVDTTQPFTVVTQFLTDDGTDTGTLSEIKRFYVQNGKVIPQPNSDIAGVTGNSITSEFCDAQKTAFGDINNFDTHGGLASMGAALQQGMVLVMSLWDDYAANMLWLDSIYPTNASASTPGAARGTCSTSSGVPSQVESQSPNAYVTYSNIKVGPINSTFTTSGSNPGGGTTTTTTTQPTTTTTTAGNPGGTGVAQHYGQCGGIGWTGPTTCASPYTCQKLNDYYSQCL

SEQ ID NO: 53 - DNA, 50 bp, Artificial Sequence
  SYNTHETIC PRIMER
caatcaactcgaccttcaccacttcgggctcgaaccctggaggcggaacg

SEQ ID NO: 54 - DNA, 34 bp, Artificial Sequence
  SYNTHETIC PRIMER
ctagatctcgagttacaaacactgcgagtagtag

SEQ ID NO: 55 - DNA, 26 bp, Artificial Sequence
  SYNTHETIC PRIMER
cgaagtggtgaaggtcgagttgattg

SEQ ID NO: 56 - DNA, 1705 bp, Artificial Sequence
  Synthetic DNA encoding a Rasamsonia byssochlamydoides cellobiohydrolase I with Aspergillus fumigatus linker and Aspergillus fumigatus carbohydrate binding module variant
  exon (1)..(603)
  sig_peptide (1)..(18)
  CDS (1)..(603)
  mat_peptide (55)..(1702)
  Intron (604)..(667)
  exon (668)..(1235)
  CDS (668)..(1235)
  Intron (1236)..(1310)
  exon (1311)..(1702)
  CDS (1311)..(1702)
atgtttcgacgggctcttttcctgtcctcttccgccttccttgctgtcaaagcccagcagatcggcacggtcagtccggagaaccatccgcccctggcatgggagcagtgcactgcccctgggagttgcacgactgtgaatggtgcggtcgtccttgatgcgaactggcgttgggtccacaatgttgggggatacaccaactgctacactggcaatacctgggacaccacgtactgccctgacgacgtgacctgcgcagagaattgtgcgctggatggcgcagattacgagggcacctacggcgtgaccacctcgggcagctccctgaagctcgatttcgtcaccgggtctaacgtcggatctcgtctctacctgttggagaatgattcgacctatcagatcttcaagcttctgaaccaggaattcacctttgacgtcgacgtttccaatcttccgtgcggattaaacggcgctctgtaccttgttaccatggctgctgacggcggggtgtctcagtacccgaataacaaggccggcgcagcgtatggaaccggttattgcgattcccagtgtccaagggacttgaagtttatcgatggccaggtatgtagagctgtaatcacccatgttgtgaaatcactctcctactgacatggtcgatttataggccaacgttgagggctggcagccgtcttcgaacaacgccaatacaggtattggcaaccatggctcctgctgtgcggagatggatatctgggaagccaacagcatctccaatgcggtgactccgcacccatgcgacacacccggccagacaatgtgcgaggggaacgactgtggtggcacgtattccaccaatcgctatgcaggcacctgcgatcctgacggctgcgacttcaacccctaccgcatgggcaaccattctttctacggccctggggagattgtcgatactacccagcccttcactgtcgtgacacagttccttaccgatgatggcacggatactggcactctcagcgagatcaaacgcttctacgtccaaaacgggaaagtcattcctcagccgaactccgacattgccggcgtgactggcaactcgatcaccagcgagttttgcgatgcccagaagacggctttcggcgacattaacaactttgatacacacggcggtctggccagtatgggagctgcgctgcagcagggtatggttctggtgatgagtctgtgggacggtaggtccttgggagacacccggacgttctatatcaaccagaactgccagaactgacgaattaaaacacttttagattacgcggcaaacatgctgtggttggacagcatttatccaacaaatgcatctgctagcactcctggtgctgctcgtggaacctgttcgacgagctccggtgtcccatcgcaagtcgagtcgcagagccccaacgcctacgtgacgtactccaacattaaagttggaccaatcaactcgaccttcaccacttcgggctcgaaccctggaggcggaacgaccactactacaacgactcagccgacaacaacaactaccacagcaggcaaccctggaggtacaggtgtggcccagcactacggacagtgtggcggtatcggatggacaggacctactacttgtgcatcgccttatacctgtcagaaattgaacgactggtactcgcagtgtttgtaa

SEQ ID NO: 57 - protein, 521 aa, Artificial Sequence
  Synthetic Construct
MFRRALFLSSSAFLAVKAQQIGTVSPENHPPLAWEQCTAPGSCTTVNGAVVLDANWRWVHNVGGYTNCYTGNTWDTTYCPDDVTCAENCALDGADYEGTYGVTTSGSSLKLDFVTGSNVGSRLYLLENDSTYQIFKLLNQEFTFDVDVSNLPCGLNGALYLVTMAADGGVSQYPNNKAGAAYGTGYCDSQCPRDLKFIDGQANVEGWQPSSNNANTGIGNHGSCCAEMDIWEANSISNAVTPHPCDTPGQTMCEGNDCGGTYSTNRYAGTCDPDGCDFNPYRMGNHSFYGPGEIVDTTQPFTVVTQFLTDDGTDTGTLSEIKRFYVQNGKVIPQPNSDIAGVTGNSITSEFCDAQKTAFGDINNFDTHGGLASMGAALQQGMVLVMSLWDDYAANMLWLDSIYPTNASASTPGAARGTCSTSSGVPSQVESQSPNAYVTYSNIKVGPINSTFTTSGSNPGGGTTTTTTTQPTTTTTTAGNPGGTGVAQHYGQCGGIGWTGPTTCASPYTCQKLNDWYSQCL

SEQ ID NO: 58 - DNA, 49 bp, Artificial Sequence
  SYNTHETIC PRIMER
atacctgtcagaaattgaacgactggtactcgcagtgtttgtaagcttc

SEQ ID NO: 59 - DNA, 32 bp, Artificial Sequence
  SYNTHETIC PRIMER
gtcgttcaatttctgacaggtataaggcgatg

SEQ ID NO: 60 - DNA, 23 bp, Artificial Sequence
  SYNTHETIC PRIMER
cctcagccgaactccgacattgc

SEQ ID NO: 61 - DNA, 23 bp, Artificial Sequence
  SYNTHETIC PRIMER
gcaatgtcggagttcggctgagg

SEQ ID NO: 62 - DNA, 1705 bp, Artificial Sequence
  Synthetic DNA encoding a Rasamsonia byssochlamydoides cellobiohydrolase I variant with Aspergillus fumigatus linker and Aspergillus fumigatus carbohydrate binding module variant
  exon (1)..(603)
  sig_peptide (1)..(18)
  CDS (1)..(603)
  mat_peptide (55)..(1702)
  Intron (604)..(667)
  exon (668)..(1235)
  CDS (668)..(1235)
  Intron (1236)..(1310)
  exon (1311)..(1702)
  CDS (1311)..(1702)
atgtttcgacgggctcttttcctgtcctcttccgccttccttgctgtcaaagcccagcagatcggcacggtcagtccggagaaccatccgcccctggcatgggagcagtgcactgcccctgggagttgcacgactgtgaatggtgcggtcgtccttgatgcgaactggcgttgggtccacaatgttgggggatacaccaactgctacactggcaatacctgggacaccacgtactgccctgacgacgtgacctgcgcagagaattgtgcgctggatggcgcagattacgagggcacctacggcgtgaccacctcgggcagctccctgaagctcgatttcgtcaccgggtctaacgtcggatctcgtctctacctgttggagaatgattcgacctatcagatcttcaagcttctgaaccaggaattcacctttgacgtcgacgtttccaatcttccgtgcggattaaacggcgctctgtaccttgttaccatggctgctgacggcggggtgtctcagtacccgaataacaaggccggcgcagcgtatggaaccggttattgcgattcccagtgtccaagggacttgaagtttatcgatggccaggtatgtagagctgtaatcacccatgttgtgaaatcactctcctactgacatggtcgatttataggccaacgttgagggctggcagccgtcttcgaacaacgccaatacaggtattggcaaccatggctcctgctgtgcggagatggatatctgggaagccaacagcatctccaatgcggtgactccgcacccatgcgacacacccggccagacaatgtgcgaggggaacgactgtggtggcacgtattccaccaatcgctatgcaggcacctgcgatcctgacggctgcgacttcaacccctaccgcatgggcaaccattctttctacggccctggggagattgtcgatactacccagcccttcacggtcgtgacacagttccttaccgatgatggcacggatactggcactctcagcgagatcaaacgcttctacgtccaaaacgggaaagtcattcctcagccgaactccgacattgccggcgtgactggcaactcgatcaccagcgagttttgcgatgcccagaagacggctttcggcgacattaacaactttgatacacacggcggtctggccagtatgggagctgcgctgcagcagggtatggttctggtgatgagtctgtgggacggtaggtccttgggagacacccggacgttctatatcaaccagaactgccagaactgacgaattaaaacacttttagattacgcggcaaacatgctgtggttggacagcatttatccaacagacgcagaccctagcactcctggtgctgctcgtggaacctgttcgacgagctccggtgtcccatcgcaagtcgagtcgcagagccccaacgcctacgtgacgtactccaacattaaagttggaccaatcaactcgaccttcaccacttcgggctcgaaccctggaggcggaacgaccactactacaacgactcagccgacaacaacaactaccacagcaggcaaccctggaggtacaggtgtggcccagcactacggacagtgtggcggtatcggatggacaggacctactacttgtgcatcgccttatacctgtcagaaattgaacgactggtactcgcagtgtttgtaa

SEQ ID NO: 63 - protein, 521 aa, Artificial Sequence
  Synthetic Construct
MFRRALFLSSSAFLAVKAQQIGTVSPENHPPLAWEQCTAPGSCTTVNGAVVLDANWRWVHNVGGYTNCYTGNTWDTTYCPDDVTCAENCALDGADYEGTYGVTTSGSSLKLDFVTGSNVGSRLYLLENDSTYQIFKLLNQEFTFDVDVSNLPCGLNGALYLVTMAADGGVSQYPNNKAGAAYGTGYCDSQCPRDLKFIDGQANVEGWQPSSNNANTGIGNHGSCCAEMDIWEANSISNAVTPHPCDTPGQTMCEGNDCGGTYSTNRYAGTCDPDGCDFNPYRMGNHSFYGPGEIVDTTQPFTVVTQFLTDDGTDTGTLSEIKRFYVQNGKVIPQPNSDIAGVTGNSITSEFCDAQKTAFGDINNFDTHGGLASMGAALQQGMVLVMSLWDDYAANMLWLDSIYPTDADPSTPGAARGTCSTSSGVPSQVESQSPNAYVTYSNIKVGPINSTFTTSGSNPGGGTTTTTTTQPTTTTTTAGNPGGTGVAQHYGQCGGIGWTGPTTCASPYTCQKLNDWYSQCL

SEQ ID NO: 64 - DNA, 55 bp, Artificial Sequence
  SYNTHETIC PRIMER
ggttggacagcatttatccaacagacgcagaccctagcactcctggtgctgctcg

SEQ ID NO: 65 - DNA, 35 bp, Artificial Sequence
  SYNTHETIC PRIMER
tgttggataaatgctgtccaaccacagcatgtttg

SEQ ID NO: 66 - DNA, 1599 bp, Aspergillus fumigatus
  sig_peptide (1)..(26)
  CDS (1)..(1596)
  mat_peptide (79)..(1596)
atgttggcctccacgttctcctatcgcatgtacaaaacagcgctcatcttggcagccctcttgggctcgggacaggcacagcaggtctgtacctcgcaggccgaggtccatccttccatgacgtggcagtcgtgtacagcgggtggttcgtgtaccacaaacaacggtaaagtcgtgatcgatgcaaactggaggtgggtgcacaaggtcggcgactacaccaactgttacacaggcaacacatgggatacaaccatctgtcccgacgatgccacttgtgcatccaactgttgtctcgagggtgccaactatgagtcgacgtacggagtgaccgcctccggaaactcgctcaggctcaacttcgtcacaacttcccagcagaagaacatcggctcgcggttgtatatgatgaaagacgattccacttacgagatgttcaagctcctcaaccaggaattcactttcgatgtcgacgtctccaacctcccttgtggcttgaacggagcgctctacttcgtcgccatggatgcggatggaggcatgtccaagtatcctaccaacaaagcaggagccaagtatggtacaggttactgtgattcccagtgtcccagggatctcaagttcatcaacggtcaggccaacgtcgagggttggcagccttcgtcgaacgatgccaacgcaggtaccggcaaccacggttcctgttgtgccgaaatggacatttgggaagcgaactcgatctcgacggcgttcactcctcacccgtgtgatacacccggacaggtgatgtgtacaggcgacgcctgtggcggaacctactcgtcggatcgatatggcggtacgtgtgaccccgacggctgtgacttcaactccttcaggcagggcaacaaaacattctatggacctggcatgacggtggatacaaagtcgaaattcacagtcgtcactcagttcatcaccgacgatggtacgtcctcgggtaccttgaaggagatcaaaaggttctatgtccagaacggaaaggtcatcccgaactcggagtccacgtggacaggagtgtcgggtaactccatcactacggagtattgtacagcccagaagtcgctcttccaggatcagaacgtcttcgagaaacatggaggcttggaaggaatgggtgccgcattggcccagggtatggtcctcgtcatgtccttgtgggacgaccactcggccaacatgctctggttggattccaactaccccaccactgcctcgtccacgacaccgggtgtcgcacgcggaacttgtgatatctcctcgggagtgcctgcagacgtcgaggcgaaccatcccgacgcctacgtggtctactcgaacattaaggtgggacccatcggttcgacattcaactccggaggctcgaaccctggaggcggaacgaccactactacaacgactcagccgacaacaacaactaccacagcaggcaaccctggaggtacaggtgtggcccagcactacggacagtgtggcggtatcggatggacaggacctactacttgtgcatcgccttatacctgtcagaaattgaacgactactactcgcagtgtttgtaa

SEQ ID NO: 67 - protein, 532 aa, Aspergillus fumigatus
MLASTFSYRMYKTALILAALLGSGQAQQVCTSQAEVHPSMTWQSCTAGGSCTTNNGKVVIDANWRWVHKVGDYTNCYTGNTWDTTICPDDATCASNCCLEGANYESTYGVTASGNSLRLNFVTTSQQKNIGSRLYMMKDDSTYEMFKLLNQEFTFDVDVSNLPCGLNGALYFVAMDADGGMSKYPTNKAGAKYGTGYCDSQCPRDLKFINGQANVEGWQPSSNDANAGTGNHGSCCAEMDIWEANSISTAFTPHPCDTPGQVMCTGDACGGTYSSDRYGGTCDPDGCDFNSFRQGNKTFYGPGMTVDTKSKFTVVTQFITDDGTSSGTLKEIKRFYVQNGKVIPNSESTWTGVSGNSITTEYCTAQKSLFQDQNVFEKHGGLEGMGAALAQGMVLVMSLWDDHSANMLWLDSNYPTTASSTTPGVARGTCDISSGVPADVEANHPDAYVVYSNIKVGPIGSTFNSGGSNPGGGTTTTTTTQPTTTTTTAGNPGGTGVAQHYGQCGGIGWTGPTTCASPYTCQKLNDYYSQCL

SEQ ID NO: 68 - DNA, 1599 bp, Aspergillus fumigatus
  sig_peptide (1)..(26)
  CDS (1)..(1596)
  mat_peptide (79)..(1596)
atgttggcctccacgttctcctatcgcatgtacaaaacagcgctcatcttggcagccctcttgggctcgggacaggcacagcaggtcggaacctcgcaggccgaggtccatccttccatgacgtggcagtcgtgtacagcgggtggttcgtgtaccacaaacaacggtaaagtcgtgatcgatgcaaactggaggtgggtgcacaagactggcgactacaccaactgttacacaggcaacacatgggatacaaccatctgtcccgacgatgccacttgtgcatccaactgtgcactcgagggtgccaactatgagtcgacgtacggagtgaccgcctccggaaactcgctcaggctcaacttcgtcacaacttcccagcagaagaacatcggctcgcggttgtatatgatgaaagacgattccacttacgagatgttcaagctcctcaaccaggaattcactttcgatgtcgacgtctccaacctcccttgtggcttgaacggagcgctctacttcgtcgccatggatgcggatggaggcatgtccaagtatcctaccaacaaagcaggagccaagtatggtacaggttactgtgattcccagtgtcccagggatctcaagttcatcaacggtcaggccaacgtcgagggttggcagccttcgtcgaacgatgccaacgcaggtaccggcaaccacggttcctgttgtgccgaaatggacatttgggaagcgaactcgatctcgacggcgttcactcctcacccgtgtgatacacccggacaggtgatgtgtacaggcgacgcctgtggcggaacctactcgtcggatcgatatggcggtacgtgtgaccccgacggctgtgacttcaaccctttcaggcagggcaacaaaacattctatggacctggcatgacggtggatacaaagtcgaaattcacagtcgtcactcagttcatcaccgacgatggtacgtcctcgggtaccttgaaggagatcaaaaggttctatgtccagaacggaaaggtcatcccgaactcggagtccacgtggacaggagtgtcgggtaactccatcactacggagtattgtacagcccagaagtcgctcttccaggatcagaacgtcttcgagaaacatggaggcttggaaggaatgggtgccgcattggcccagggtatggtcctcgtcatgtccttgtgggacgaccactcggccaacatgctctggttggattccaactaccccaccactgcctcgtccacgacaccgggtgtcgcacgcggaacttgtgatatctcctcgggagtgcctgcagacgtcgaggcgaaccatcccgacgcctacgtggtctactcgaacattaaggtgggacccatcggttcgacattcaactccggaggctcgaaccctggaggcggaacgaccactactacaacgactcagccgacaacaacaactaccacagcaggcaaccctggaggtacaggtgtggcccagcactacggacagtgtggcggtatcggatggacaggacctactacttgtgcatcgccttatacctgtcagaaattgaacgactactactcgcagtgtttgtaa

SEQ ID NO: 69 - protein, 532 aa, Aspergillus fumigatus
MLASTFSYRMYKTALILAALLGSGQAQQVGTSQAEVHPSMTWQSCTAGGSCTTNNGKVVIDANWRWVHKTGDYTNCYTGNTWDTTICPDDATCASNCALEGANYESTYGVTASGNSLRLNFVTTSQQKNIGSRLYMMKDDSTYEMFKLLNQEFTFDVDVSNLPCGLNGALYFVAMDADGGMSKYPTNKAGAKYGTGYCDSQCPRDLKFINGQANVEGWQPSSNDANAGTGNHGSCCAEMDIWEANSISTAFTPHPCDTPGQVMCTGDACGGTYSSDRYGGTCDPDGCDFNPFRQGNKTFYGPGMTVDTKSKFTVVTQFITDDGTSSGTLKEIKRFYVQNGKVIPNSESTWTGVSGNSITTEYCTAQKSLFQDQNVFEKHGGLEGMGAALAQGMVLVMSLWDDHSANMLWLDSNYPTTASSTTPGVARGTCDISSGVPADVEANHPDAYVVYSNIKVGPIGSTFNSGGSNPGGGTTTTTTTQPTTTTTTAGNPGGTGVAQHYGQCGGIGWTGPTTCASPYTCQKLNDYYSQCL

SEQ ID NO: 70 - DNA, 1599 bp, Aspergillus fumigatus
  sig_peptide (1)..(26)
  CDS (1)..(1596)
  mat_peptide (79)..(1596)
atgttggcctccacgttctcctatcgcatgtacaaaacagcgctcatcttggcagccctcttgggctcgggacaggcacagcaggtcggaacctcgcaggccgaggtccatccttccatgacgtggcagtcgtgtacagcgggtggttcgtgtaccacaaacaacggtaaagtcgtgatcgatgcaaactggaggtgggtgcacaaggtcggcgactacaccaactgttacacaggcaacacatgggatacaaccatctgtcccgacgatgccacttgtgcatccaactgtgcactcgagggtgccaactatgagtcgacgtacggagtgaccgcctccggaaactcgctcaggctcaacttcgtcacaacttcccagcagaagaacatcggctcgcggttgtatatgatgaaagacgattccacttacgagatgttcaagctcctcaaccaggaattcactttcgatgtcgacgtctccaacctcccttgtggcttgaacggagcgctctacttcgtcgccatggatgcggatggaggcatgtccaagtatcctaccaacaaagcaggagccaagtatggtacaggttactgtgattcccagtgtcccagggatctcaagttcatcaacggtcaggccaacgtcgagggttggcagccttcgtcgaacgatgccaacgcaggtaccggcaaccacggttcctgttgtgccgaaatggacatttgggaagcgaactcgatctcgacggcgttcactcctcacccgtgtgatacacccggacaggtgatgtgtacaggcgacgcctgtggcggaacctactcgtcggatcgatatggcggtacgtgtgaccccgacggctgtgacttcaactccttcaggcagggcaacaaaacattctatggacctggcatgacggtggatacaaagtcgaaattcacagtcgtcactcagttcatcaccgacgatggtacgtcctcgggtaccttgaaggagatcaaaaggttctatgtccagaacggaaaggtcatcccgaactcggagtccacgtggacaggagtgtcgggtaactccatcactacggagtattgtacagcccagaagtcgctcttccaggatcagaacgtcttcgagaaacatggaggcttggaaggaatgggtgccgcattggcccagggtatggtcctcgtcatgtccttgtgggacgaccactcggccaacatgctctggttggattccaactaccccaccactgccgatcctacgacaccgggtgtcgcacgcggaacttgtgatatctcctcgggagtgcctgcagacgtcgaggcgaaccatcccgacgcctacgtggtctactcgaacattaaggtgggacccatcggttcgacattcaactccggaggctcgaaccctggaggcggaacgaccactactacaacgactcagccgacaacaacaactaccacagcaggcaaccctggaggtacaggtgtggcccagcactacggacagtgtggcggtatcggatggacaggacctactacttgtgcatcgccttatacctgtcagaaattgaacgactactactcgcagtgtttgtaa

SEQ ID NO: 71 - protein, 532 aa, Aspergillus fumigatus
MLASTFSYRMYKTALILAALLGSGQAQQVGTSQAEVHPSMTWQSCTAGGSCTTNNGKVVIDANWRWVHKVGDYTNCYTGNTWDTTICPDDATCASNCALEGANYESTYGVTASGNSLRLNFVTTSQQKNIGSRLYMMKDDSTYEMFKLLNQEFTFDVDVSNLPCGLNGALYFVAMDADGGMSKYPTNKAGAKYGTGYCDSQCPRDLKFINGQANVEGWQPSSNDANAGTGNHGSCCAEMDIWEANSISTAFTPHPCDTPGQVMCTGDACGGTYSSDRYGGTCDPDGCDFNSFRQGNKTFYGPGMTVDTKSKFTVVTQFITDDGTSSGTLKEIKRFYVQNGKVIPNSESTWTGVSGNSITTEYCTAQKSLFQDQNVFEKHGGLEGMGAALAQGMVLVMSLWDDHSANMLWLDSNYPTTADPTTPGVARGTCDISSGVPADVEANHPDAYVVYSNIKVGPIGSTFNSGGSNPGGGTTTTTTTQPTTTTTTAGNPGGTGVAQHYGQCGGIGWTGPTTCASPYTCQKLNDYYSQCL

SEQ ID NO: 72 - DNA, 1599 bp, Aspergillus fumigatus
  sig_peptide (1)..(26)
  CDS (1)..(1596)
  mat_peptide (79)..(1596)
atgttggcctccacgttctcctatcgcatgtacaaaacagcgctcatcttggcagccctcttgggctcgggacaggcacagcaggtcggaacctcgcaggccgaggtccatccttccatgacgtggcagtcgtgtacagcgggtggttcgtgtaccacaaacaacggtaaagtcgtgatcgatgcaaactggaggtgggtgcacaagatcggcgactacaccaactgttacacaggcaacacatgggatacaaccatctgtcccgacgatgccacttgtgcatccaactgtgcactcgagggtgccaactatgagtcgacgtacggagtgaccgcctccggaaactcgctcaggctcaacttcgtcacaacttcccagcagaagaacatcggctcgcggttgtatatgatgaaagacgattccacttacgagatgttcaagctcctcaaccaggaattcactttcgatgtcgacgtctccaacctcccttgtggcttgaacggagcgctctacttcgtcgccatggatgcggatggaggcatgtccaagtatcctaccaacaaagcaggagccaagtatggtacaggttactgtgattcccagtgtcccagggatctcaagttcatcaacggtcaggccaacgtcgagggttggcagccttcgtcgaacgatgccaacgcaggtaccggcaaccacggttcctgttgtgccgaaatggacatttgggaagcgaactcgatctcgacggcgttcactcctcacccgtgtgatacacccggacaggtgatgtgtacaggcgacgcctgtggcggaacctactcgtcggatcgatatggcggtacgtgtgaccccgacggctgtgacttcaactccttcaggcagggcaacaaaacattctatggacctggcatgacggtggatacaaagtcgaaattcacagtcgtcactcagttcatcaccgacgatggtacgtcctcgggtaccttgaaggagatcaaaaggttctatgtccagaacggaaaggtcatcccgaactcggagtccacgtggacaggagtgtcgggtaactccatcactacggagtattgtacagcccagaagtcgctcttccaggatcagaacgtcttcgagaaacatggaggcttggaaggaatgggtgccgcattggcccagggtatggtcctcgtcatgtccttgtgggacgaccactcggccaacatgctctggttggattccaactaccccaccactgcctcgtccacgacaccgggtgtcgcacgcggaacttgtgatatctcctcgggagtgcctgcagacgtcgaggcgaaccatcccgacgcctacgtggtctactcgaacattaaggtgggacccatcggttcgacattcaactccggaggctcgaaccctggaggcggaacgaccactactacaacgactcagccgacaacaacaactaccacagcaggcaaccctggaggtacaggtgtggcccagcactacggacagtgtggcggtatcggatggacaggacctactacttgtgcatcgccttatacctgtcagaaattgaacgactactactcgcagtgtttgtaa

SEQ ID NO: 73 - protein, 532 aa, Aspergillus fumigatus
MLASTFSYRMYKTALILAALLGSGQAQQVGTSQAEVHPSMTWQSCTAGGSCTTNNGKVVIDANWRWVHKIGDYTNCYTGNTWDTTICPDDATCASNCALEGANYESTYGVTASGNSLRLNFVTTSQQKNIGSRLYMMKDDSTYEMFKLLNQEFTFDVDVSNLPCGLNGALYFVAMDADGGMSKYPTNKAGAKYGTGYCDSQCPRDLKFINGQANVEGWQPSSNDANAGTGNHGSCCAEMDIWEANSISTAFTPHPCDTPGQVMCTGDACGGTYSSDRYGGTCDPDGCDFNSFRQGNKTFYGPGMTVDTKSKFTVVTQFITDDGTSSGTLKEIKRFYVQNGKVIPNSESTWTGVSGNSITTEYCTAQKSLFQDQNVFEKHGGLEGMGAALAQGMVLVMSLWDDHSANMLWLDSNYPTTASSTTPGVARGTCDISSGVPADVEANHPDAYVVYSNIKVGPIGSTFNSGGSNPGGGTTTTTTTQPTTTTTTAGNPGGTGVAQHYGQCGGIGWTGPTTCASPYTCQKLNDYYSQCL

SEQ ID NO: 74 - DNA, 1599 bp, Aspergillus fumigatus
  sig_peptide (1)..(26)
  CDS (1)..(1596)
  mat_peptide (79)..(1596)
atgttggcctccacgttctcctatcgcatgtacaaaacagcgctcatcttggcagccctcttgggctcgggacaggcacagcaggtcggaacctcgcaggccgaggtccatccttccatgacgtggcagtcgtgtacagcgggtggttcgtgtaccacaaacaacggtaaagtcgtgatcgatgcaaactggaggtgggtgcacaagatgggcgactacaccaactgttacacaggcaacacatgggatacaaccatctgtcccgacgatgccacttgtgcatccaactgtgcactcgagggtgccaactatgagtcgacgtacggagtgaccgcctccggaaactcgctcaggctcaacttcgtcacaacttcccagcagaagaacatcggctcgcggttgtatatgatgaaagacgattccacttacgagatgttcaagctcctcaaccaggaattcactttcgatgtcgacgtctccaacctcccttgtggcttgaacggagcgctctacttcgtcgccatggatgcggatggaggcatgtccaagtatcctaccaacaaagcaggagccaagtatggtacaggttactgtgattcccagtgtcccagggatctcaagttcatcaacggtcaggccaacgtcgagggttggcagccttcgtcgaacgatgccaacgcaggtaccggcaaccacggttcctgttgtgccgaaatggacatttgggaagcgaactcgatctcgacggcgttcactcctcacccgtgtgatacacccggacaggtgatgtgtacaggcgacgcctgtggcggaacctactcgtcggatcgatatggcggtacgtgtgaccccgacggctgtgacttcaactccttcaggcagggcaacaaaacattctatggacctggcatgacggtggatacaaagtcgaaattcacagtcgtcactcagttcatcaccgacgatggtacgtcctcgggtaccttgaaggagatcaaaaggttctatgtccagaacggaaaggtcatcccgaactcggagtccacgtggacaggagtgtcgggtaactccatcactacggagtattgtacagcccagaagtcgctcttccaggatcagaacgtcttcgagaaacatggaggcttggaaggaatgggtgccgcattggcccagggtatggtcctcgtcatgtccttgtgggacgaccactcggccaacatgctctggttggattccaactaccccaccactgcctcgtccacgacaccgggtgtcgcacgcggaacttgtgatatctcctcgggagtgcctgcagacgtcgaggcgaaccatcccgacgcctacgtggtctactcgaacattaaggtgggacccatcggttcgacattcaactccggaggctcgaaccctggaggcggaacgaccactactacaacgactcagccgacaacaacaactaccacagcaggcaaccctggaggtacaggtgtggcccagcactacggacagtgtggcggtatcggatggacaggacctactacttgtgcatcgccttatacctgtcagaaattgaacgactactactcgcagtgtttgtaa

SEQ ID NO: 75 - protein, 532 aa, Aspergillus fumigatus
MLASTFSYRMYKTALILAALLGSGQAQQVGTSQAEVHPSMTWQSCTAGGSCTTNNGKVVIDANWRWVHKMGDYTNCYTGNTWDTTICPDDATCASNCALEGANYESTYGVTASGNSLRLNFVTTSQQKNIGSRLYMMKDDSTYEMFKLLNQEFTFDVDVSNLPCGLNGALYFVAMDADGGMSKYPTNKAGAKYGTGYCDSQCPRDLKFINGQANVEGWQPSSNDANAGTGNHGSCCAEMDIWEANSISTAFTPHPCDTPGQVMCTGDACGGTYSSDRYGGTCDPDGCDFNSFRQGNKTFYGPGMTVDTKSKFTVVTQFITDDGTSSGTLKEIKRFYVQNGKVIPNSESTWTGVSGNSITTEYCTAQKSLFQDQNVFEKHGGLEGMGAALAQGMVLVMSLWDDHSANMLWLDSNYPTTASSTTPGVARGTCDISSGVPADVEANHPDAYVVYSNIKVGPIGSTFNSGGSNPGGGTTTTTTTQPTTTTTTAGNPGGTGVAQHYGQCGGIGWTGPTTCASPYTCQKLNDYYSQCL

SEQ ID NO: 76 - DNA, 1599 bp, Aspergillus fumigatus
  sig_peptide (1)..(26)
  CDS (1)..(1596)
  mat_peptide (79)..(1596)
atgttggcctccacgttctcctatcgcatgtacaaaacagcgctcatcttggcagccctcttgggctcgggacaggcacagcaggtcggaacctcgcaggccgaggtccatccttccatgacgtggcagtcgtgtacagcgggtggttcgtgtaccacaaacaacggtaaagtcgtgatcgatgcaaactggaggtgggtgcacaagaacggcgactacaccaactgttacacaggcaacacatgggatacaaccatctgtcccgacgatgccacttgtgcatccaactgtgcactcgagggtgccaactatgagtcgacgtacggagtgaccgcctccggaaactcgctcaggctcaacttcgtcacaacttcccagcagaagaacatcggctcgcggttgtatatgatgaaagacgattccacttacgagatgttcaagctcctcaaccaggaattcactttcgatgtcgacgtctccaacctcccttgtggcttgaacggagcgctctacttcgtcgccatggatgcggatggaggcatgtccaagtatcctaccaacaaagcaggagccaagtatggtacaggttactgtgattcccagtgtcccagggatctcaagttcatcaacggtcaggccaacgtcgagggttggcagccttcgtcgaacgatgccaacgcaggtaccggcaaccacggttcctgttgtgccgaaatggacatttgggaagcgaactcgatctcgacggcgttcactcctcacccgtgtgatacacccggacaggtgatgtgtacaggcgacgcctgtggcggaacctactcgtcggatcgatatggcggtacgtgtgaccccgacggctgtgacttcaactccttcaggcagggcaacaaaacattctatggacctggcatgacggtggatacaaagtcgaaattcacagtcgtcactcagttcatcaccgacgatggtacgtcctcgggtaccttgaaggagatcaaaaggttctatgtccagaacggaaaggtcatcccgaactcggagtccacgtggacaggagtgtcgggtaactccatcactacggagtattgtacagcccagaagtcgctcttccaggatcagaacgtcttcgagaaacatggaggcttggaaggaatgggtgccgcattggcccagggtatggtcctcgtcatgtccttgtgggacgaccactcggccaacatgctctggttggattccaactaccccaccactgcctcgtccacgacaccgggtgtcgcacgcggaacttgtgatatctcctcgggagtgcctgcagacgtcgaggcgaaccatcccgacgcctacgtggtctactcgaacattaaggtgggacccatcggttcgacattcaactccggaggctcgaaccctggaggcggaacgaccactactacaacgactcagccgacaacaacaactaccacagcaggcaaccctggaggtacaggtgtggcccagcactacggacagtgtggcggtatcggatggacaggacctactacttgtgcatcgccttatacctgtcagaaattgaacgactactactcgcagtgtttgtaa

SEQ ID NO: 77 - protein, 532 aa, Aspergillus fumigatus
MLASTFSYRMYKTALILAALLGSGQAQQVGTSQAEVHPSMTWQSCTAGGSCTTNNGKVVIDANWRWVHKNGDYTNCYTGNTWDTTICPDDATCASNCALEGANYESTYGVTASGNSLRLNFVTTSQQKNIGSRLYMMKDDSTYEMFKLLNQEFTFDVDVSNLPCGLNGALYFVAMDADGGMSKYPTNKAGAKYGTGYCDSQCPRDLKFINGQANVEGWQPSSNDANAGTGNHGSCCAEMDIWEANSISTAFTPHPCDTPGQVMCTGDACGGTYSSDRYGGTCDPDGCDFNSFRQGNKTFYGPGMTVDTKSKFTVVTQFITDDGTSSGTLKEIKRFYVQNGKVIPNSESTWTGVSGNSITTEYCTAQKSLFQDQNVFEKHGGLEGMGAALAQGMVLVMSLWDDHSANMLWLDSNYPTTASSTTPGVARGTCDISSGVPADVEANHPDAYVVYSNIKVGPIGSTFNSGGSNPGGGTTTTTTTQPTTTTTTAGNPGGTGVAQHYGQCGGIGWTGPTTCASPYTCQKLNDYYSQCL

SEQ ID NO: 78 - DNA, 1599 bp, Aspergillus fumigatus
  sig_peptide (1)..(26)
  CDS (1)..(1596)
  mat_peptide (79)..(1596)
atgttggcctccacgttctcctatcgcatgtacaaaacagcgctcatcttggcagccctcttgggctcgggacaggcacagcaggtcggaacctcgcaggccgaggtccatccttccatgacgtggcagtcgtgtacagcgggtggttcgtgtaccacaaacaacggtaaagtcgtgatcgatgcaaactggaggtgggtgcacaagaagggcgactacaccaactgttacacaggcaacacatgggatacaaccatctgtcccgacgatgccacttgtgcatccaactgtgcactcgagggtgccaactatgagtcgacgtacggagtgaccgcctccggaaactcgctcaggctcaacttcgtcacaacttcccagcagaagaacatcggctcgcggttgtatatgatgaaagacgattccacttacgagatgttcaagctcctcaaccaggaattcactttcgatgtcgacgtctccaacctcccttgtggcttgaacggagcgctctacttcgtcgccatggatgcggatggaggcatgtccaagtatcctaccaacaaagcaggagccaagtatggtacaggttactgtgattcccagtgtcccagggatctcaagttcatcaacggtcaggccaacgtcgagggttggcagccttcgtcgaacgatgccaacgcaggtaccggcaaccacggttcctgttgtgccgaaatggacatttgggaagcgaactcgatctcgacggcgttcactcctcacccgtgtgatacacccggacaggtgatgtgtacaggcgacgcctgtggcggaacctactcgtcggatcgatatggcggtacgtgtgaccccgacggctgtgacttcaactccttcaggcagggcaacaaaacattctatggacctggcatgacggtggatacaaagtcgaaattcacagtcgtcactcagttcatcaccgacgatggtacgtcctcgggtaccttgaaggagatcaaaaggttctatgtccagaacggaaaggtcatcccgaactcggagtccacgtggacaggagtgtcgggtaactccatcactacggagtattgtacagcccagaagtcgctcttccaggatcagaacgtcttcgagaaacatggaggcttggaaggaatgggtgccgcattggcccagggtatggtcctcgtcatgtccttgtgggacgaccactcggccaacatgctctggttggattccaactaccccaccactgcctcgtccacgacaccgggtgtcgcacgcggaacttgtgatatctcctcgggagtgcctgcagacgtcgaggcgaaccatcccgacgcctacgtggtctactcgaacattaaggtgggacccatcggttcgacattcaactccggaggctcgaaccctggaggcggaacgaccactactacaacgactcagccgacaacaacaactaccacagcaggcaaccctggaggtacaggtgtggcccagcactacggacagtgtggcggtatcggatggacaggacctactacttgtgcatcgccttatacctgtcagaaattgaacgactactactcgcagtgtttgtaa

SEQ ID NO: 79 - protein, 532 aa, Aspergillus fumigatus
MLASTFSYRMYKTALILAALLGSGQAQQVGTSQAEVHPSMTWQSCTAGGSCTTNNGKVVIDANWRWVHKKGDYTNCYTGNTWDTTICPDDATCASNCALEGANYESTYGVTASGNSLRLNFVTTSQQKNIGSRLYMMKDDSTYEMFKLLNQEFTFDVDVSNLPCGLNGALYFVAMDADGGMSKYPTNKAGAKYGTGYCDSQCPRDLKFINGQANVEGWQPSSNDANAGTGNHGSCCAEMDIWEANSISTAFTPHPCDTPGQVMCTGDACGGTYSSDRYGGTCDPDGCDFNSFRQGNKTFYGPGMTVDTKSKFTVVTQFITDDGTSSGTLKEIKRFYVQNGKVIPNSESTWTGVSGNSITTEYCTAQKSLFQDQNVFEKHGGLEGMGAALAQGMVLVMSLWDDHSANMLWLDSNYPTTASSTTPGVARGTCDISSGVPADVEANHPDAYVVYSNIKVGPIGSTFNSGGSNPGGGTTTTTTTQPTTTTTTAGNPGGTGVAQHYGQCGGIGWTGPTTCASPYTCQKLNDYYSQCL

SEQ ID NO: 80 - DNA, 1599 bp, Aspergillus fumigatus
  sig_peptide (1)..(26)
  CDS (1)..(1596)
  mat_peptide (79)..(1596)
atgttggcctccacgttctcctatcgcatgtacaaaacagcgctcatcttggcagccctcttgggctcgggacaggcacagcaggtcggaacctcgcaggccgaggtccatccttccatgacgtggcagtcgtgtacagcgggtggttcgtgtaccacaaacaacggtaaagtcgtgatcgatgcaaactggaggtgggtgcacaaggtcggcgactacaccaactgttacacaggcaacacatgggatacaaccatctgtcccgacgatgccacttgtgcatccaactgtgcactcgagggtgccaactatgagtcgacgtacggagtgaccgcctccggaaactcgctcaggctcaacttcgtcacaacttcccagcagaagaacatcggctcgcggttgtatatgatgaaagacgattccacttacgagatgttcaagctcctcaaccaggaattcactttcgatgtcgacgtctccaacctcccttgtggcttgaacggagcgctctacttcgtcgccatggatgcggatggaggcatgtccaagtatcctaccaacaaagcaggagccaagtatggtacaggttactgtgattcccagtgtcccagggatctcaagttcatcaacggtcaggccaacgtcgagggttggcagccttcgtcgaacgatgccaacgcaggtaccggcaaccacggttcctgttgtgccgaaatggacatttgggaagcgaactcgatctcgacggcgttcactcctcacccgtgtgatacacccggacaggtgatgtgtacaggcgacgcctgtggcggaacctactcgtcggatcgatatggcggtacgtgtgaccccgacggctgtgacttcaactccttcaggcagggcaacaaaacattctatggacctggcatgacggtggatacaaagtcgaaattcacagtcgtcactcagttcatcaccgacgatggtacgtcctcgggtaccttgaaggagatcaaaaggttctatgtccagaacggaaaggtcatcccgaactcggagtccacgtggacaggagtgtcgggtaactccatcactacggagtattgtacagcccagaagtcgctcttccaggatcagaacgtcttcgagaaacatggaggcttggaaggaatgggtgccgcattggcccagggtatggtcctcgtcatgtccttgtgggacgaccactcggccaacatgctctggttggattccaactaccccacctgggccgatcctacgacaccgggtgtcgcacgcggaacttgtgatatctcctcgggagtgcctgcagacgtcgaggcgaaccatcccgacgcctacgtggtctactcgaacattaaggtgggacccatcggttcgacattcaactccggaggctcgaaccctggaggcggaacgaccactactacaacgactcagccgacaacaacaactaccacagcaggcaaccctggaggtacaggtgtggcccagcactacggacagtgtggcggtatcggatggacaggacctactacttgtgcatcgccttatacctgtcagaaattgaacgactactactcgcagtgtttgtaa

SEQ ID NO: 81 - protein, 532 aa, Aspergillus fumigatus
MLASTFSYRMYKTALILAALLGSGQAQQVGTSQAEVHPSMTWQSCTAGGSCTTNNGKVVIDANWRWVHKVGDYTNCYTGNTWDTTICPDDATCASNCALEGANYESTYGVTASGNSLRLNFVTTSQQKNIGSRLYMMKDDSTYEMFKLLNQEFTFDVDVSNLPCGLNGALYFVAMDADGGMSKYPTNKAGAKYGTGYCDSQCPRDLKFINGQANVEGWQPSSNDANAGTGNHGSCCAEMDIWEANSISTAFTPHPCDTPGQVMCTGDACGGTYSSDRYGGTCDPDGCDFNSFRQGNKTFYGPGMTVDTKSKFTVVTQFITDDGTSSGTLKEIKRFYVQNGKVIPNSESTWTGVSGNSITTEYCTAQKSLFQDQNVFEKHGGLEGMGAALAQGMVLVMSLWDDHSANMLWLDSNYPTWADPTTPGVARGTCDISSGVPADVEANHPDAYVVYSNIKVGPIGSTFNSGGSNPGGGTTTTTTTQPTTTTTTAGNPGGTGVAQHYGQCGGIGWTGPTTCASPYTCQKLNDYYSQCL

SEQ ID NO: 82 - DNA, 1599 bp, Aspergillus fumigatus
  sig_peptide (1)..(26)
  CDS (1)..(1596)
  mat_peptide (79)..(1596)
atgttggcctccacgttctcctatcgcatgtacaaaacagcgctcatcttggcagccctcttgggctcgggacaggcacagcaggtcggaacctcgcaggccgaggtccatccttccatgacgtggcagtcgtgtacagcgggtggttcgtgtaccacaaacaacggtaaagtcgtgatcgatgcaaactggaggtgggtgcacaaggtcggcgactacaccaactgttacacaggcaacacatgggatacaaccatctgtcccgacgatgccacttgtgcatccaactgtgcactcgagggtgccaactatgagtcgacgtacggagtgaccgcctccggaaactcgctcaggctcaacttcgtcacaacttcccagcagaagaacatcggctcgcggttgtatatgatgaaagacgattccacttacgagatgttcaagctcctcaaccaggaattcactttcgatgtcgacgtctccaacctcccttgtggcttgaacggagcgctctacttcgtcgccatggatgcggatggaggcatgtccaagtatcctaccaacaaagcaggagccaagtatggtacaggttactgtgattcccagtgtcccagggatctcaagttcatcaacggtcaggccaacgtcgagggttggcagccttcgtcgaacgatgccaacgcaggtaccggcaaccacggttcctgttgtgccgaaatggacatttgggaagcgaactcgatctcgacggcgttcactcctcacccgtgtgatacacccggacaggtgatgtgtacaggcgacgcctgtggcggaacctactcgtcggatcgatatggcggtacgtgtgaccccgacggctgtgacttcaactccttcaggcagggcaacaaaacattctatggacctggcatgacggtggatacaaagtcgaaattcacagtcgtcactcagttcatcaccgacgatggtacgtcctcgggtaccttgaaggagatcaaaaggttctatgtccagaacggaaaggtcatcccgaactcggagtccacgtggacaggagtgtcgggtaactccatcactacggagtattgtacagcccagaagtcgctcttccaggatcagaacgtcttcgagaaacatggaggcttggaaggaatgggtgccgcattggcccagggtatggtcctcgtcatgtccttgtgggacgaccactcggccaacatgctctggttggattccaactaccccaccgtcgccgatcctacgacaccgggtgtcgcacgcggaacttgtgatatctcctcgggagtgcctgcagacgtcgaggcgaaccatcccgacgcctacgtggtctactcgaacattaaggtgggacccatcggttcgacattcaactccggaggctcgaaccctggaggcggaacgaccactactacaacgactcagccgacaacaacaactaccacagcaggcaaccctggaggtacaggtgtggcccagcactacggacagtgtggcggtatcggatggacaggacctactacttgtgcatcgccttatacctgtcagaaattgaacgactactactcgcagtgtttgtaa

SEQ ID NO: 83 - protein, 532 aa, Aspergillus fumigatus
MLASTFSYRMYKTALILAALLGSGQAQQVGTSQAEVHPSMTWQSCTAGGSCTTNNGKVVIDANWRWVHKVGDYTNCYTGNTWDTTICPDDATCASNCALEGANYESTYGVTASGNSLRLNFVTTSQQKNIGSRLYMMKDDSTYEMFKLLNQEFTFDVDVSNLPCGLNGALYFVAMDADGGMSKYPTNKAGAKYGTGYCDSQCPRDLKFINGQANVEGWQPSSNDANAGTGNHGSCCAEMDIWEANSISTAFTPHPCDTPGQVMCTGDACGGTYSSDRYGGTCDPDGCDFNSFRQGNKTFYGPGMTVDTKSKFTVVTQFITDDGTSSGTLKEIKRFYVQNGKVIPNSESTWTGVSGNSITTEYCTAQKSLFQDQNVFEKHGGLEGMGAALAQGMVLVMSLWDDHSANMLWLDSNYPTVADPTTPGVARGTCDISSGVPADVEANHPDAYVVYSNIKVGPIGSTFNSGGSNPGGGTTTTTTTQPTTTTTTAGNPGGTGVAQHYGQCGGIGWTGPTTCASPYTCQKLNDYYSQCL

SEQ ID NO: 84 - DNA, 1599 bp, Aspergillus fumigatus
  sig_peptide (1)..(26)
  CDS (1)..(1596)
  mat_peptide (79)..(1596)
atgttggcctccacgttctcctatcgcatgtacaaaacagcgctcatcttggcagccctcttgggctcgggacaggcacagcaggtcggaacctcgcaggccgaggtccatccttccatgacgtggcagtcgtgtacagcgggtggttcgtgtaccacaaacaacggtaaagtcgtgatcgatgcaaactggaggtgggtgcacaaggtcggcgactacaccaactgttacacaggcaacacatgggatacaaccatctgtcccgacgatgccacttgtgcatccaactgtgcactcgagggtgccaactatgagtcgacgtacggagtgaccgcctccggaaactcgctcaggctcaacttcgtcacaacttcccagcagaagaacatcggctcgcggttgtatatgatgaaagacgattccacttacgagatgttcaagctcctcaaccaggaattcactttcgatgtcgacgtctccaacctcccttgtggcttgaacggagcgctctacttcgtcgccatggatgcggatggaggcatgtccaagtatcctaccaacaaagcaggagccaagtatggtacaggttactgtgattcccagtgtcccagggatctcaagttcatcaacggtcaggccaacgtcgagggttggcagccttcgtcgaacgatgccaacgcaggtaccggcaaccacggttcctgttgtgccgaaatggacatttgggaagcgaactcgatctcgacggcgttcactcctcacccgtgtgatacacccggacaggtgatgtgtacaggcgacgcctgtggcggaacctactcgtcggatcgatatggcggtacgtgtgaccccgacggctgtgacttcaactccttcaggcagggcaacaaaacattctatggacctggcatgacggtggatacaaagtcgaaattcacagtcgtcactcagttcatcaccgacgatggtacgtcctcgggtaccttgaaggagatcaaaaggttctatgtccagaacggaaaggtcatcccgaactcggagtccacgtggacaggagtgtcgggtaactccatcactacggagtattgtacagcccagaagtcgctcttccaggatcagaacgtcttcgagaaacatggaggcttggaaggaatgggtgccgcattggcccagggtatggtcctcgtcatgtccttgtgggacgaccactcggccaacatgctctggttggattccaactaccccaccaacgccgatcctacgacaccgggtgtcgcacgcggaacttgtgatatctcctcgggagtgcctgcagacgtcgaggcgaaccatcccgacgcctacgtggtctactcgaacattaaggtgggacccatcggttcgacattcaactccggaggctcgaaccctggaggcggaacgaccactactacaacgactcagccgacaacaacaactaccacagcaggcaaccctggaggtacaggtgtggcccagcactacggacagtgtggcggtatcggatggacaggacctactacttgtgcatcgccttatacctgtcagaaattgaacgactactactcgcagtgtttgtaa

SEQ ID NO: 85 - protein, 532 aa, Aspergillus fumigatus
MLASTFSYRMYKTALILAALLGSGQAQQVGTSQAEVHPSMTWQSCTAGGSCTTNNGKVVIDANWRWVHKVGDYTNCYTGNTWDTTICPDDATCASNCALEGANYESTYGVTASGNSLRLNFVTTSQQKNIGSRLYMMKDDSTYEMFKLLNQEFTFDVDVSNLPCGLNGALYFVAMDADGGMSKYPTNKAGAKYGTGYCDSQCPRDLKFINGQANVEGWQPSSNDANAGTGNHGSCCAEMDIWEANSISTAFTPHPCDTPGQVMCTGDACGGTYSSDRYGGTCDPDGCDFNSFRQGNKTFYGPGMTVDTKSKFTVVTQFITDDGTSSGTLKEIKRFYVQNGKVIPNSESTWTGVSGNSITTEYCTAQKSLFQDQNVFEKHGGLEGMGAALAQGMVLVMSLWDDHSANMLWLDSNYPTNADPTTPGVARGTCDISSGVPADVEANHPDAYVVYSNIKVGPIGSTFNSGGSNPGGGTTTTTTTQPTTTTTTAGNPGGTGVAQHYGQCGGIGWTGPTTCASPYTCQKLNDYYSQCL